European Patent Application EP 4 316 586 A2, published February 7, 2024. Title: TOXIN-DERIVED DELIVERY CONSTRUCTS. Applicant: APPLIED MOLECULAR TRANSPORT INC. Application EP. The sequence listing filed with the application follows.

SEQUENCE LISTING (221 sequences)

SEQ ID NO: 1 - protein, 634 aa, Vibrio cholera
VEEALNIFDECRSPCSLTPEPGKPIQSKLSIPSDVVLDEGVLYYSMTINDEQNDIKDEDKGESIITIGEFATVRATRHYVNQDAPFGVIHLDITTENGTKTYSYNRKEGEFAINWLVPIGEDSPASIKISVDELDQQRNIIEVPKLYSIDLDNQTLEQWKTQGNVSFSVTRPEHNIAISWPSVSYKAAQKEGSRHKRWAHWHTGLALCWLVPMDAIYNYITQQNCTLGDNWFGGSYETVAGTPKVITVKQGIEQKPVEQRIHFSKGNAMSALAAHRVCGVPLETLARSRKPRDLTDDLSCAYQAQNIVSLFVATRILFSHLDSVFTLNLDEQEPEVAERLSDLRRINENNPGMVTQVLTVARQIYNDYVTHHPGLTPEQTSAGAQAADILSLFCPDADKSCVASNNDQANINIESRSGRSYLPENRAVITPQGVTNWTYQELEATHQALTREGYVFVGYHGTNHVAAQTIVNRIAPVPRGNNTENEEKWGGLYVATHAEVAHGYARIKEGTGEYGLPTRAERDARGVMLRVYIPRASLERFYRTNTPLENAEEHITQVIGHSLPLRNEAFTGPESAGGEDETVIGWDMAIHAVAIPSTIPGNAYEELAIDEEAVAKEQSISTKPPYKERKDELK

SEQ ID NO: 2 - protein, 634 aa, Vibrio cholera
VEDELNIFDECRSPCSLTPEPGKPIQSKLSIPSDVVLDEGVLYYSMTINDEQNDIKDEDKGESIITIGEFATVRATRHYVNQDAPFGVIHLDITTENGTKTYSYNRKEGEFAINWLVPIGEDSPASIKISVDELDQQRNIIEVPKLYSIDLDNQTLEQWKTQGNVSFSVTRPEHNIAISWPSVSYKAAQKEGSRHKRWAHWHTGLALCWLVPMDAIYNYITQQNCTLGDNWFGGSYETVAGTPKVITVKQGIEQKPVEQRIHFSKGNAMSALAAHRVCGVPLETLARSRKPRDLTDDLSCAYQAQNIVSLFVATRILFSHLDSVFTLNLDEQEPEVAERLSDLRRINENNPGMVTQVLTVARQIYNDYVTHHPGLTPEQTSAGAQAADILSLFCPDADKSCVASNNDQANINIESRSGRSYLPENRAVITPQGVTNWTYQELEATHQALTREGYVFVGYHGTNHVAAQTIVNRIAPVPRGNNTENEEKWGGLYVATHAEVAHGYARIKEGTGEYGLPTRAERDARGVMLRVYIPRASLERFYRTNTPLENAEEHITQVIGHSLPLRNEAFTGPESAGGEDETVIGWDMAIHAVAIPSTIPGNAYEELAIDEEAVAKEQSISTKPPYKERKDELK

SEQ ID NO: 3 - protein, 634 aa, Vibrio cholera
VEDELNIFDECRSPCSLTPEPGKPIQSKLSIPSDVVLDEGVLYYSMTINDEQNDIKDEDKGESIITIGEFATVRATRHYVNQDAPFGVIHLDITTENGTKTYSYNRKEGEFAINWLVPIGEDSPASIKISVDELDQQRNIIEVPKLYSIDLDNQTLEQWKTQGNVSFSVTRPEHNIAISWPSVSYKAAQKEGSRHKRWAHWHTGLALCWLVPMDAIYNYITQQNCTLGDNWFGGSYETVAGTPKVITVKQGIEQKPVEQRIHFSKGNAMSALAAHRVCGVPLETLARSRKPRDLTDDLSCAYQAQNIVSLFVATRILFSHLDSVFTLNLDEQEPEVAERLSDLRRINENNPGMVTQVLTVARQIYNDYVTHHPGLTPEQTSAGAQAADILSLFCPDADKSCVASNNDQANINIESRSGRSYLPENRAVITPQGVTNWTYQELEATHQALTREGYVFVGYHGTNHVAAQTIVNRIAPVPRGNNTENEEKWGGLYVATHAEVAHGYARIKEGTGEYGLPTRAERDARGVMLRVYIPRASLERFYRTNTPLENAEEHITQVIGHSLPLRNEAFTGPESAGGEDATVIGWDMAIHAVAIPSTIPGNAYEELAIDEEAVAKEQSISTKPPYKERKDELK

SEQ ID NO: 4 - protein, 265 aa, Vibrio cholera
VEEALNIFDECRSPCSLTPEPGKPIQSKLSIPSDVVLDEGVLYYSMTINDEQNDIKDEDKGESIITIGEFATVRATRHYVNQDAPFGVIHLDITTENGTKTYSYNRKEGEFAINWLVPIGEDSPASIKISVDELDQQRNIIEVPKLYSIDLDNQTLEQWKTQGNVSFSVTRPEHNIAISWPSVSYKAAQKEGSRHKRWAHWHTGLALCWLVPMDAIYNYITQQNCTLGDNWFGGSYETVAGTPKVITVKQGIEQKPVEQRIHFSK

SEQ ID NO: 5 - protein, 266 aa, synthetic construct
  source 1..266: note = Description of Artificial Sequence: Synthetic polypeptide
MVEEALNIFDECRSPCSLTPEPGKPIQSKLSIPSDVVLDEGVLYYSMTINDEQNDIKDEDKGESIITIGEFATVRATRHYVNQDAPFGVIHLDITTENGTKTYSYNRKEGEFAINWLVPIGEDSPASIKISVDELDQQRNIIEVPKLYSIDLDNQTLEQWKTQGNVSFSVTRPEHNIAISWPSVSYKAAQKEGSRHKRWAHWHTGLALCWLVPMDAIYNYITQQNCTLGDNWFGGSYETVAGTPKVITVKQGIEQKPVEQRIHFSK

SEQ ID NO: 6 - protein, 250 aa, Vibrio cholera
VEEALNIFDECRSPCSLTPEPGKPIQSKLSIPSDVVLDEGVLYYSMTINDEQNDIKDEDKGESIITIGEFATVRATRHYVNQDAPFGVIHLDITTENGTKTYSYNRKEGEFAINWLVPIGEDSPASIKISVDELDQQRNIIEVPKLYSIDLDNQTLEQWKTQGNVSFSVTRPEHNIAISWPSVSYKAAQKEGSRHKRWAHWHTGLALCWLVPMDAIYNYITQQNCTLGDNWFGGSYETVAGTPKVITVKQ

SEQ ID NO: 7 - protein, 251 aa, synthetic construct
  source 1..251: note = Description of Artificial Sequence: Synthetic polypeptide
MVEEALNIFDECRSPCSLTPEPGKPIQSKLSIPSDVVLDEGVLYYSMTINDEQNDIKDEDKGESIITIGEFATVRATRHYVNQDAPFGVIHLDITTENGTKTYSYNRKEGEFAINWLVPIGEDSPASIKISVDELDQQRNIIEVPKLYSIDLDNQTLEQWKTQGNVSFSVTRPEHNIAISWPSVSYKAAQKEGSRHKRWAHWHTGLALCWLVPMDAIYNYITQQNCTLGDNWFGGSYETVAGTPKVITVKQ

SEQ ID NO: 8 - protein, 244 aa, Vibrio cholera
VEEALNIFDECRSPCSLTPEPGKPIQSKLSIPSDVVLDEGVLYYSMTINDEQNDIKDEDKGESIITIGEFATVRATRHYVNQDAPFGVIHLDITTENGTKTYSYNRKEGEFAINWLVPIGEDSPASIKISVDELDQQRNIIEVPKLYSIDLDNQTLEQWKTQGNVSFSVTRPEHNIAISWPSVSYKAAQKEGSRHKRWAHWHTGLALCWLVPMDAIYNYITQQNCTLGDNWFGGSYETVAGTPK

SEQ ID NO: 9 - protein, 245 aa, synthetic construct
  source 1..245: note = Description of Artificial Sequence: Synthetic polypeptide
MVEEALNIFDECRSPCSLTPEPGKPIQSKLSIPSDVVLDEGVLYYSMTINDEQNDIKDEDKGESIITIGEFATVRATRHYVNQDAPFGVIHLDITTENGTKTYSYNRKEGEFAINWLVPIGEDSPASIKISVDELDQQRNIIEVPKLYSIDLDNQTLEQWKTQGNVSFSVTRPEHNIAISWPSVSYKAAQKEGSRHKRWAHWHTGLALCWLVPMDAIYNYITQQNCTLGDNWFGGSYETVAGTPK

SEQ ID NO: 10 - protein, 205 aa, Vibrio cholera
VEEALNIFDECRSPCSLTPEPGKPIQSKLSIPSDVVLDEGVLYYSMTINDEQNDIKDEDKGESIITIGEFATVRATRHYVNQDAPFGVIHLDITTENGTKTYSYNRKEGEFAINWLVPIGEDSPASIKISVDELDQQRNIIEVPKLYSIDLDNQTLEQWKTQGNVSFSVTRPEHNIAISWPSVSYKAAQKEGSRHKRWAHWHTGL

SEQ ID NO: 11 - protein, 206 aa, synthetic construct
  source 1..206: note = Description of Artificial Sequence: Synthetic polypeptide
MVEEALNIFDECRSPCSLTPEPGKPIQSKLSIPSDVVLDEGVLYYSMTINDEQNDIKDEDKGESIITIGEFATVRATRHYVNQDAPFGVIHLDITTENGTKTYSYNRKEGEFAINWLVPIGEDSPASIKISVDELDQQRNIIEVPKLYSIDLDNQTLEQWKTQGNVSFSVTRPEHNIAISWPSVSYKAAQKEGSRHKRWAHWHTGL

SEQ ID NO: 12 - protein, 204 aa, Vibrio cholera
VEEALNIFDECRSPCSLTPEPGKPIQSKLSIPSDVVLDEGVLYYSMTINDEQNDIKDEDKGESIITIGEFATVRATRHYVNQDAPFGVIHLDITTENGTKTYSYNRKEGEFAINWLVPIGEDSPASIKISVDELDQQRNIIEVPKLYSIDLDNQTLEQWKTQGNVSFSVTRPEHNIAISWPSVSYKAAQKEGSRHKRWAHWHTG

SEQ ID NO: 13 - protein, 203 aa, Vibrio cholera
VEEALNIFDECRSPCSLTPEPGKPIQSKLSIPSDVVLDEGVLYYSMTINDEQNDIKDEDKGESIITIGEFATVRATRHYVNQDAPFGVIHLDITTENGTKTYSYNRKEGEFAINWLVPIGEDSPASIKISVDELDQQRNIIEVPKLYSIDLDNQTLEQWKTQGNVSFSVTRPEHNIAISWPSVSYKAAQKEGSRHKRWAHWHT

SEQ ID NO: 14 - protein, 202 aa, Vibrio cholera
VEEALNIFDECRSPCSLTPEPGKPIQSKLSIPSDVVLDEGVLYYSMTINDEQNDIKDEDKGESIITIGEFATVRATRHYVNQDAPFGVIHLDITTENGTKTYSYNRKEGEFAINWLVPIGEDSPASIKISVDELDQQRNIIEVPKLYSIDLDNQTLEQWKTQGNVSFSVTRPEHNIAISWPSVSYKAAQKEGSRHKRWAHWH

SEQ ID NO: 15 - protein, 201 aa, Vibrio cholera
VEEALNIFDECRSPCSLTPEPGKPIQSKLSIPSDVVLDEGVLYYSMTINDEQNDIKDEDKGESIITIGEFATVRATRHYVNQDAPFGVIHLDITTENGTKTYSYNRKEGEFAINWLVPIGEDSPASIKISVDELDQQRNIIEVPKLYSIDLDNQTLEQWKTQGNVSFSVTRPEHNIAISWPSVSYKAAQKEGSRHKRWAHW

SEQ ID NO: 16 - protein, 200 aa, Vibrio cholera
VEEALNIFDECRSPCSLTPEPGKPIQSKLSIPSDVVLDEGVLYYSMTINDEQNDIKDEDKGESIITIGEFATVRATRHYVNQDAPFGVIHLDITTENGTKTYSYNRKEGEFAINWLVPIGEDSPASIKISVDELDQQRNIIEVPKLYSIDLDNQTLEQWKTQGNVSFSVTRPEHNIAISWPSVSYKAAQKEGSRHKRWAH

SEQ ID NO: 17 - protein, 199 aa, Vibrio cholera
VEEALNIFDECRSPCSLTPEPGKPIQSKLSIPSDVVLDEGVLYYSMTINDEQNDIKDEDKGESIITIGEFATVRATRHYVNQDAPFGVIHLDITTENGTKTYSYNRKEGEFAINWLVPIGEDSPASIKISVDELDQQRNIIEVPKLYSIDLDNQTLEQWKTQGNVSFSVTRPEHNIAISWPSVSYKAAQKEGSRHKRWA

SEQ ID NO: 18 - protein, 198 aa, Vibrio cholera
VEEALNIFDECRSPCSLTPEPGKPIQSKLSIPSDVVLDEGVLYYSMTINDEQNDIKDEDKGESIITIGEFATVRATRHYVNQDAPFGVIHLDITTENGTKTYSYNRKEGEFAINWLVPIGEDSPASIKISVDELDQQRNIIEVPKLYSIDLDNQTLEQWKTQGNVSFSVTRPEHNIAISWPSVSYKAAQKEGSRHKRW

SEQ ID NO: 19 - protein, 197 aa, Vibrio cholera
VEEALNIFDECRSPCSLTPEPGKPIQSKLSIPSDVVLDEGVLYYSMTINDEQNDIKDEDKGESIITIGEFATVRATRHYVNQDAPFGVIHLDITTENGTKTYSYNRKEGEFAINWLVPIGEDSPASIKISVDELDQQRNIIEVPKLYSIDLDNQTLEQWKTQGNVSFSVTRPEHNIAISWPSVSYKAAQKEGSRHKR

SEQ ID NO: 20 - protein, 196 aa, Vibrio cholera
VEEALNIFDECRSPCSLTPEPGKPIQSKLSIPSDVVLDEGVLYYSMTINDEQNDIKDEDKGESIITIGEFATVRATRHYVNQDAPFGVIHLDITTENGTKTYSYNRKEGEFAINWLVPIGEDSPASIKISVDELDQQRNIIEVPKLYSIDLDNQTLEQWKTQGNVSFSVTRPEHNIAISWPSVSYKAAQKEGSRHK

SEQ ID NO: 21 - protein, 195 aa, Vibrio cholera
VEEALNIFDECRSPCSLTPEPGKPIQSKLSIPSDVVLDEGVLYYSMTINDEQNDIKDEDKGESIITIGEFATVRATRHYVNQDAPFGVIHLDITTENGTKTYSYNRKEGEFAINWLVPIGEDSPASIKISVDELDQQRNIIEVPKLYSIDLDNQTLEQWKTQGNVSFSVTRPEHNIAISWPSVSYKAAQKEGSRH

SEQ ID NO: 22 - protein, 194 aa, Vibrio cholera
VEEALNIFDECRSPCSLTPEPGKPIQSKLSIPSDVVLDEGVLYYSMTINDEQNDIKDEDKGESIITIGEFATVRATRHYVNQDAPFGVIHLDITTENGTKTYSYNRKEGEFAINWLVPIGEDSPASIKISVDELDQQRNIIEVPKLYSIDLDNQTLEQWKTQGNVSFSVTRPEHNIAISWPSVSYKAAQKEGSR

SEQ ID NO: 23 - protein, 193 aa, Vibrio cholera
VEEALNIFDECRSPCSLTPEPGKPIQSKLSIPSDVVLDEGVLYYSMTINDEQNDIKDEDKGESIITIGEFATVRATRHYVNQDAPFGVIHLDITTENGTKTYSYNRKEGEFAINWLVPIGEDSPASIKISVDELDQQRNIIEVPKLYSIDLDNQTLEQWKTQGNVSFSVTRPEHNIAISWPSVSYKAAQKEGS

SEQ ID NO: 24 - protein, 192 aa, Vibrio cholera
VEEALNIFDECRSPCSLTPEPGKPIQSKLSIPSDVVLDEGVLYYSMTINDEQNDIKDEDKGESIITIGEFATVRATRHYVNQDAPFGVIHLDITTENGTKTYSYNRKEGEFAINWLVPIGEDSPASIKISVDELDQQRNIIEVPKLYSIDLDNQTLEQWKTQGNVSFSVTRPEHNIAISWPSVSYKAAQKEG

SEQ ID NO: 25 - protein, 191 aa, Vibrio cholera
VEEALNIFDECRSPCSLTPEPGKPIQSKLSIPSDVVLDEGVLYYSMTINDEQNDIKDEDKGESIITIGEFATVRATRHYVNQDAPFGVIHLDITTENGTKTYSYNRKEGEFAINWLVPIGEDSPASIKISVDELDQQRNIIEVPKLYSIDLDNQTLEQWKTQGNVSFSVTRPEHNIAISWPSVSYKAAQKE

SEQ ID NO: 26 - protein, 190 aa, Vibrio cholera
VEEALNIFDECRSPCSLTPEPGKPIQSKLSIPSDVVLDEGVLYYSMTINDEQNDIKDEDKGESIITIGEFATVRATRHYVNQDAPFGVIHLDITTENGTKTYSYNRKEGEFAINWLVPIGEDSPASIKISVDELDQQRNIIEVPKLYSIDLDNQTLEQWKTQGNVSFSVTRPEHNIAISWPSVSYKAAQK

SEQ ID NO: 27 - protein, 189 aa, Vibrio cholera
VEEALNIFDECRSPCSLTPEPGKPIQSKLSIPSDVVLDEGVLYYSMTINDEQNDIKDEDKGESIITIGEFATVRATRHYVNQDAPFGVIHLDITTENGTKTYSYNRKEGEFAINWLVPIGEDSPASIKISVDELDQQRNIIEVPKLYSIDLDNQTLEQWKTQGNVSFSVTRPEHNIAISWPSVSYKAAQ

SEQ ID NO: 28 - protein, 188 aa, Vibrio cholera
VEEALNIFDECRSPCSLTPEPGKPIQSKLSIPSDVVLDEGVLYYSMTINDEQNDIKDEDKGESIITIGEFATVRATRHYVNQDAPFGVIHLDITTENGTKTYSYNRKEGEFAINWLVPIGEDSPASIKISVDELDQQRNIIEVPKLYSIDLDNQTLEQWKTQGNVSFSVTRPEHNIAISWPSVSYKAA

SEQ ID NO: 29 - protein, 187 aa, Vibrio cholera
VEEALNIFDECRSPCSLTPEPGKPIQSKLSIPSDVVLDEGVLYYSMTINDEQNDIKDEDKGESIITIGEFATVRATRHYVNQDAPFGVIHLDITTENGTKTYSYNRKEGEFAINWLVPIGEDSPASIKISVDELDQQRNIIEVPKLYSIDLDNQTLEQWKTQGNVSFSVTRPEHNIAISWPSVSYKA

SEQ ID NO: 30 - protein, 186 aa, Vibrio cholera
VEEALNIFDECRSPCSLTPEPGKPIQSKLSIPSDVVLDEGVLYYSMTINDEQNDIKDEDKGESIITIGEFATVRATRHYVNQDAPFGVIHLDITTENGTKTYSYNRKEGEFAINWLVPIGEDSPASIKISVDELDQQRNIIEVPKLYSIDLDNQTLEQWKTQGNVSFSVTRPEHNIAISWPSVSYK

SEQ ID NO: 31 - protein, 187 aa, synthetic construct
  source 1..187: note = Description of Artificial Sequence: Synthetic polypeptide
MVEEALNIFDECRSPCSLTPEPGKPIQSKLSIPSDVVLDEGVLYYSMTINDEQNDIKDEDKGESIITIGEFATVRATRHYVNQDAPFGVIHLDITTENGTKTYSYNRKEGEFAINWLVPIGEDSPASIKISVDELDQQRNIIEVPKLYSIDLDNQTLEQWKTQGNVSFSVTRPEHNIAISWPSVSYK

SEQ ID NO: 32 - protein, 185 aa, Vibrio cholera
EEALNIFDECRSPCSLTPEPGKPIQSKLSIPSDVVLDEGVLYYSMTINDEQNDIKDEDKGESIITIGEFATVRATRHYVNQDAPFGVIHLDITTENGTKTYSYNRKEGEFAINWLVPIGEDSPASIKISVDELDQQRNIIEVPKLYSIDLDNQTLEQWKTQGNVSFSVTRPEHNIAISWPSVSYK

SEQ ID NO: 33 - protein, 184 aa, Vibrio cholera
EALNIFDECRSPCSLTPEPGKPIQSKLSIPSDVVLDEGVLYYSMTINDEQNDIKDEDKGESIITIGEFATVRATRHYVNQDAPFGVIHLDITTENGTKTYSYNRKEGEFAINWLVPIGEDSPASIKISVDELDQQRNIIEVPKLYSIDLDNQTLEQWKTQGNVSFSVTRPEHNIAISWPSVSYK

SEQ ID NO: 34 - protein, 183 aa, Vibrio cholera
ALNIFDECRSPCSLTPEPGKPIQSKLSIPSDVVLDEGVLYYSMTINDEQNDIKDEDKGESIITIGEFATVRATRHYVNQDAPFGVIHLDITTENGTKTYSYNRKEGEFAINWLVPIGEDSPASIKISVDELDQQRNIIEVPKLYSIDLDNQTLEQWKTQGNVSFSVTRPEHNIAISWPSVSYK

SEQ ID NO: 35 - protein, 182 aa, Vibrio cholera
LNIFDECRSPCSLTPEPGKPIQSKLSIPSDVVLDEGVLYYSMTINDEQNDIKDEDKGESIITIGEFATVRATRHYVNQDAPFGVIHLDITTENGTKTYSYNRKEGEFAINWLVPIGEDSPASIKISVDELDQQRNIIEVPKLYSIDLDNQTLEQWKTQGNVSFSVTRPEHNIAISWPSVSYK

SEQ ID NO: 36 - protein, 181 aa, Vibrio cholera
NIFDECRSPCSLTPEPGKPIQSKLSIPSDVVLDEGVLYYSMTINDEQNDIKDEDKGESIITIGEFATVRATRHYVNQDAPFGVIHLDITTENGTKTYSYNRKEGEFAINWLVPIGEDSPASIKISVDELDQQRNIIEVPKLYSIDLDNQTLEQWKTQGNVSFSVTRPEHNIAISWPSVSYK

SEQ ID NO: 37 - protein, 180 aa, Vibrio cholera
IFDECRSPCSLTPEPGKPIQSKLSIPSDVVLDEGVLYYSMTINDEQNDIKDEDKGESIITIGEFATVRATRHYVNQDAPFGVIHLDITTENGTKTYSYNRKEGEFAINWLVPIGEDSPASIKISVDELDQQRNIIEVPKLYSIDLDNQTLEQWKTQGNVSFSVTRPEHNIAISWPSVSYK

SEQ ID NO: 38 - protein, 179 aa, Vibrio cholera
FDECRSPCSLTPEPGKPIQSKLSIPSDVVLDEGVLYYSMTINDEQNDIKDEDKGESIITIGEFATVRATRHYVNQDAPFGVIHLDITTENGTKTYSYNRKEGEFAINWLVPIGEDSPASIKISVDELDQQRNIIEVPKLYSIDLDNQTLEQWKTQGNVSFSVTRPEHNIAISWPSVSYK

SEQ ID NO: 39 - protein, 178 aa, Vibrio cholera
DECRSPCSLTPEPGKPIQSKLSIPSDVVLDEGVLYYSMTINDEQNDIKDEDKGESIITIGEFATVRATRHYVNQDAPFGVIHLDITTENGTKTYSYNRKEGEFAINWLVPIGEDSPASIKISVDELDQQRNIIEVPKLYSIDLDNQTLEQWKTQGNVSFSVTRPEHNIAISWPSVSYK

SEQ ID NO: 40 - protein, 177 aa, Vibrio cholera
ECRSPCSLTPEPGKPIQSKLSIPSDVVLDEGVLYYSMTINDEQNDIKDEDKGESIITIGEFATVRATRHYVNQDAPFGVIHLDITTENGTKTYSYNRKEGEFAINWLVPIGEDSPASIKISVDELDQQRNIIEVPKLYSIDLDNQTLEQWKTQGNVSFSVTRPEHNIAISWPSVSYK

SEQ ID NO: 41 - protein, 176 aa, Vibrio cholera
CRSPCSLTPEPGKPIQSKLSIPSDVVLDEGVLYYSMTINDEQNDIKDEDKGESIITIGEFATVRATRHYVNQDAPFGVIHLDITTENGTKTYSYNRKEGEFAINWLVPIGEDSPASIKISVDELDQQRNIIEVPKLYSIDLDNQTLEQWKTQGNVSFSVTRPEHNIAISWPSVSYK

SEQ ID NO: 42 - protein, 175 aa, Vibrio cholera
RSPCSLTPEPGKPIQSKLSIPSDVVLDEGVLYYSMTINDEQNDIKDEDKGESIITIGEFATVRATRHYVNQDAPFGVIHLDITTENGTKTYSYNRKEGEFAINWLVPIGEDSPASIKISVDELDQQRNIIEVPKLYSIDLDNQTLEQWKTQGNVSFSVTRPEHNIAISWPSVSYK

SEQ ID NO: 43 - protein, 174 aa, Vibrio cholera
SPCSLTPEPGKPIQSKLSIPSDVVLDEGVLYYSMTINDEQNDIKDEDKGESIITIGEFATVRATRHYVNQDAPFGVIHLDITTENGTKTYSYNRKEGEFAINWLVPIGEDSPASIKISVDELDQQRNIIEVPKLYSIDLDNQTLEQWKTQGNVSFSVTRPEHNIAISWPSVSYK

SEQ ID NO: 44 - protein, 173 aa, Vibrio cholera
PCSLTPEPGKPIQSKLSIPSDVVLDEGVLYYSMTINDEQNDIKDEDKGESIITIGEFATVRATRHYVNQDAPFGVIHLDITTENGTKTYSYNRKEGEFAINWLVPIGEDSPASIKISVDELDQQRNIIEVPKLYSIDLDNQTLEQWKTQGNVSFSVTRPEHNIAISWPSVSYK

SEQ ID NO: 45 - protein, 172 aa, Vibrio cholera
CSLTPEPGKPIQSKLSIPSDVVLDEGVLYYSMTINDEQNDIKDEDKGESIITIGEFATVRATRHYVNQDAPFGVIHLDITTENGTKTYSYNRKEGEFAINWLVPIGEDSPASIKISVDELDQQRNIIEVPKLYSIDLDNQTLEQWKTQGNVSFSVTRPEHNIAISWPSVSYK

SEQ ID NO: 46 - protein, 171 aa, Vibrio cholera
SLTPEPGKPIQSKLSIPSDVVLDEGVLYYSMTINDEQNDIKDEDKGESIITIGEFATVRATRHYVNQDAPFGVIHLDITTENGTKTYSYNRKEGEFAINWLVPIGEDSPASIKISVDELDQQRNIIEVPKLYSIDLDNQTLEQWKTQGNVSFSVTRPEHNIAISWPSVSYK

SEQ ID NO: 47 - protein, 170 aa, Vibrio cholera
LTPEPGKPIQSKLSIPSDVVLDEGVLYYSMTINDEQNDIKDEDKGESIITIGEFATVRATRHYVNQDAPFGVIHLDITTENGTKTYSYNRKEGEFAINWLVPIGEDSPASIKISVDELDQQRNIIEVPKLYSIDLDNQTLEQWKTQGNVSFSVTRPEHNIAISWPSVSYK

SEQ ID NO: 48 - protein, 169 aa, Vibrio cholera
TPEPGKPIQSKLSIPSDVVLDEGVLYYSMTINDEQNDIKDEDKGESIITIGEFATVRATRHYVNQDAPFGVIHLDITTENGTKTYSYNRKEGEFAINWLVPIGEDSPASIKISVDELDQQRNIIEVPKLYSIDLDNQTLEQWKTQGNVSFSVTRPEHNIAISWPSVSYK

SEQ ID NO: 49 - protein, 168 aa, Vibrio cholera
PEPGKPIQSKLSIPSDVVLDEGVLYYSMTINDEQNDIKDEDKGESIITIGEFATVRATRHYVNQDAPFGVIHLDITTENGTKTYSYNRKEGEFAINWLVPIGEDSPASIKISVDELDQQRNIIEVPKLYSIDLDNQTLEQWKTQGNVSFSVTRPEHNIAISWPSVSYK

SEQ ID NO: 50 - protein, 167 aa, Vibrio cholera
EPGKPIQSKLSIPSDVVLDEGVLYYSMTINDEQNDIKDEDKGESIITIGEFATVRATRHYVNQDAPFGVIHLDITTENGTKTYSYNRKEGEFAINWLVPIGEDSPASIKISVDELDQQRNIIEVPKLYSIDLDNQTLEQWKTQGNVSFSVTRPEHNIAISWPSVSYK

SEQ ID NO: 51 - protein, 166 aa, Vibrio cholera
PGKPIQSKLSIPSDVVLDEGVLYYSMTINDEQNDIKDEDKGESIITIGEFATVRATRHYVNQDAPFGVIHLDITTENGTKTYSYNRKEGEFAINWLVPIGEDSPASIKISVDELDQQRNIIEVPKLYSIDLDNQTLEQWKTQGNVSFSVTRPEHNIAISWPSVSYK

SEQ ID NO: 52 - protein, 165 aa, Vibrio cholera
GKPIQSKLSIPSDVVLDEGVLYYSMTINDEQNDIKDEDKGESIITIGEFATVRATRHYVNQDAPFGVIHLDITTENGTKTYSYNRKEGEFAINWLVPIGEDSPASIKISVDELDQQRNIIEVPKLYSIDLDNQTLEQWKTQGNVSFSVTRPEHNIAISWPSVSYK

SEQ ID NO: 53 - protein, 164 aa, Vibrio cholera
KPIQSKLSIPSDVVLDEGVLYYSMTINDEQNDIKDEDKGESIITIGEFATVRATRHYVNQDAPFGVIHLDITTENGTKTYSYNRKEGEFAINWLVPIGEDSPASIKISVDELDQQRNIIEVPKLYSIDLDNQTLEQWKTQGNVSFSVTRPEHNIAISWPSVSYK

SEQ ID NO: 54 - protein, 163 aa, Vibrio cholera
PIQSKLSIPSDVVLDEGVLYYSMTINDEQNDIKDEDKGESIITIGEFATVRATRHYVNQDAPFGVIHLDITTENGTKTYSYNRKEGEFAINWLVPIGEDSPASIKISVDELDQQRNIIEVPKLYSIDLDNQTLEQWKTQGNVSFSVTRPEHNIAISWPSVSYK

SEQ ID NO: 55 - protein, 162 aa, Vibrio cholera
IQSKLSIPSDVVLDEGVLYYSMTINDEQNDIKDEDKGESIITIGEFATVRATRHYVNQDAPFGVIHLDITTENGTKTYSYNRKEGEFAINWLVPIGEDSPASIKISVDELDQQRNIIEVPKLYSIDLDNQTLEQWKTQGNVSFSVTRPEHNIAISWPSVSYK

SEQ ID NO: 56 - protein, 161 aa, Vibrio cholera
QSKLSIPSDVVLDEGVLYYSMTINDEQNDIKDEDKGESIITIGEFATVRATRHYVNQDAPFGVIHLDITTENGTKTYSYNRKEGEFAINWLVPIGEDSPASIKISVDELDQQRNIIEVPKLYSIDLDNQTLEQWKTQGNVSFSVTRPEHNIAISWPSVSYK

SEQ ID NO: 57 - protein, 160 aa, Vibrio cholera
SKLSIPSDVVLDEGVLYYSMTINDEQNDIKDEDKGESIITIGEFATVRATRHYVNQDAPFGVIHLDITTENGTKTYSYNRKEGEFAINWLVPIGEDSPASIKISVDELDQQRNIIEVPKLYSIDLDNQTLEQWKTQGNVSFSVTRPEHNIAISWPSVSYK

SEQ ID NO: 58 - protein, 159 aa, Vibrio cholera
KLSIPSDVVLDEGVLYYSMTINDEQNDIKDEDKGESIITIGEFATVRATRHYVNQDAPFGVIHLDITTENGTKTYSYNRKEGEFAINWLVPIGEDSPASIKISVDELDQQRNIIEVPKLYSIDLDNQTLEQWKTQGNVSFSVTRPEHNIAISWPSVSYK

SEQ ID NO: 59 - protein, 158 aa, Vibrio cholera
LSIPSDVVLDEGVLYYSMTINDEQNDIKDEDKGESIITIGEFATVRATRHYVNQDAPFGVIHLDITTENGTKTYSYNRKEGEFAINWLVPIGEDSPASIKISVDELDQQRNIIEVPKLYSIDLDNQTLEQWKTQGNVSFSVTRPEHNIAISWPSVSYK

SEQ ID NO: 60 - protein, 157 aa, Vibrio cholera
SIPSDVVLDEGVLYYSMTINDEQNDIKDEDKGESIITIGEFATVRATRHYVNQDAPFGVIHLDITTENGTKTYSYNRKEGEFAINWLVPIGEDSPASIKISVDELDQQRNIIEVPKLYSIDLDNQTLEQWKTQGNVSFSVTRPEHNIAISWPSVSYK

SEQ ID NO: 61 - protein, 156 aa, Vibrio cholera
IPSDVVLDEGVLYYSMTINDEQNDIKDEDKGESIITIGEFATVRATRHYVNQDAPFGVIHLDITTENGTKTYSYNRKEGEFAINWLVPIGEDSPASIKISVDELDQQRNIIEVPKLYSIDLDNQTLEQWKTQGNVSFSVTRPEHNIAISWPSVSYK

SEQ ID NO: 62 - protein, 155 aa, Vibrio cholera
PSDVVLDEGVLYYSMTINDEQNDIKDEDKGESIITIGEFATVRATRHYVNQDAPFGVIHLDITTENGTKTYSYNRKEGEFAINWLVPIGEDSPASIKISVDELDQQRNIIEVPKLYSIDLDNQTLEQWKTQGNVSFSVTRPEHNIAISWPSVSYK

SEQ ID NO: 63 - protein, 154 aa, Vibrio cholera
SDVVLDEGVLYYSMTINDEQNDIKDEDKGESIITIGEFATVRATRHYVNQDAPFGVIHLDITTENGTKTYSYNRKEGEFAINWLVPIGEDSPASIKISVDELDQQRNIIEVPKLYSIDLDNQTLEQWKTQGNVSFSVTRPEHNIAISWPSVSYK

SEQ ID NO: 64 - protein, 153 aa, Vibrio cholera
DVVLDEGVLYYSMTINDEQNDIKDEDKGESIITIGEFATVRATRHYVNQDAPFGVIHLDITTENGTKTYSYNRKEGEFAINWLVPIGEDSPASIKISVDELDQQRNIIEVPKLYSIDLDNQTLEQWKTQGNVSFSVTRPEHNIAISWPSVSYK

SEQ ID NO: 65 - protein, 152 aa, Vibrio cholera
VVLDEGVLYYSMTINDEQNDIKDEDKGESIITIGEFATVRATRHYVNQDAPFGVIHLDITTENGTKTYSYNRKEGEFAINWLVPIGEDSPASIKISVDELDQQRNIIEVPKLYSIDLDNQTLEQWKTQGNVSFSVTRPEHNIAISWPSVSYK

SEQ ID NO: 66 - protein, 151 aa, Vibrio cholera
VLDEGVLYYSMTINDEQNDIKDEDKGESIITIGEFATVRATRHYVNQDAPFGVIHLDITTENGTKTYSYNRKEGEFAINWLVPIGEDSPASIKISVDELDQQRNIIEVPKLYSIDLDNQTLEQWKTQGNVSFSVTRPEHNIAISWPSVSYK

SEQ ID NO: 67 - protein, 150 aa, Vibrio cholera
LDEGVLYYSMTINDEQNDIKDEDKGESIITIGEFATVRATRHYVNQDAPFGVIHLDITTENGTKTYSYNRKEGEFAINWLVPIGEDSPASIKISVDELDQQRNIIEVPKLYSIDLDNQTLEQWKTQGNVSFSVTRPEHNIAISWPSVSYK

SEQ ID NO: 68 - protein, 149 aa, Vibrio cholera
DEGVLYYSMTINDEQNDIKDEDKGESIITIGEFATVRATRHYVNQDAPFGVIHLDITTENGTKTYSYNRKEGEFAINWLVPIGEDSPASIKISVDELDQQRNIIEVPKLYSIDLDNQTLEQWKTQGNVSFSVTRPEHNIAISWPSVSYK

SEQ ID NO: 69 - protein, 148 aa, Vibrio cholera
EGVLYYSMTINDEQNDIKDEDKGESIITIGEFATVRATRHYVNQDAPFGVIHLDITTENGTKTYSYNRKEGEFAINWLVPIGEDSPASIKISVDELDQQRNIIEVPKLYSIDLDNQTLEQWKTQGNVSFSVTRPEHNIAISWPSVSYK

SEQ ID NO: 70 - protein, 147 aa, Vibrio cholera
GVLYYSMTINDEQNDIKDEDKGESIITIGEFATVRATRHYVNQDAPFGVIHLDITTENGTKTYSYNRKEGEFAINWLVPIGEDSPASIKISVDELDQQRNIIEVPKLYSIDLDNQTLEQWKTQGNVSFSVTRPEHNIAISWPSVSYK

SEQ ID NO: 71 - protein, 185 aa, Vibrio cholera
VEEALNIFDECRSPCSLTPEPGKPIQSKLSIPSDVVLDEGVLYYSMTINDEQNDIKDEDKGESIITIGEFATVRATRHYVNQDAPFGVIHLDITTENGTKTYSYNRKEGEFAINWLVPIGEDSPASIKISVDELDQQRNIIEVPKLYSIDLDNQTLEQWKTQGNVSFSVTRPEHNIAISWPSVSY

SEQ ID NO: 72 - protein, 184 aa, Vibrio cholera
VEEALNIFDECRSPCSLTPEPGKPIQSKLSIPSDVVLDEGVLYYSMTINDEQNDIKDEDKGESIITIGEFATVRATRHYVNQDAPFGVIHLDITTENGTKTYSYNRKEGEFAINWLVPIGEDSPASIKISVDELDQQRNIIEVPKLYSIDLDNQTLEQWKTQGNVSFSVTRPEHNIAISWPSVS

SEQ ID NO: 73 - protein, 183 aa, Vibrio cholera
VEEALNIFDECRSPCSLTPEPGKPIQSKLSIPSDVVLDEGVLYYSMTINDEQNDIKDEDKGESIITIGEFATVRATRHYVNQDAPFGVIHLDITTENGTKTYSYNRKEGEFAINWLVPIGEDSPASIKISVDELDQQRNIIEVPKLYSIDLDNQTLEQWKTQGNVSFSVTRPEHNIAISWPSV

SEQ ID NO: 74 - protein, 182 aa, Vibrio cholera
VEEALNIFDECRSPCSLTPEPGKPIQSKLSIPSDVVLDEGVLYYSMTINDEQNDIKDEDKGESIITIGEFATVRATRHYVNQDAPFGVIHLDITTENGTKTYSYNRKEGEFAINWLVPIGEDSPASIKISVDELDQQRNIIEVPKLYSIDLDNQTLEQWKTQGNVSFSVTRPEHNIAISWPS

SEQ ID NO: 75 - protein, 181 aa, Vibrio cholera
VEEALNIFDECRSPCSLTPEPGKPIQSKLSIPSDVVLDEGVLYYSMTINDEQNDIKDEDKGESIITIGEFATVRATRHYVNQDAPFGVIHLDITTENGTKTYSYNRKEGEFAINWLVPIGEDSPASIKISVDELDQQRNIIEVPKLYSIDLDNQTLEQWKTQGNVSFSVTRPEHNIAISWP

SEQ ID NO: 76 - protein, 180 aa, Vibrio cholera
VEEALNIFDECRSPCSLTPEPGKPIQSKLSIPSDVVLDEGVLYYSMTINDEQNDIKDEDKGESIITIGEFATVRATRHYVNQDAPFGVIHLDITTENGTKTYSYNRKEGEFAINWLVPIGEDSPASIKISVDELDQQRNIIEVPKLYSIDLDNQTLEQWKTQGNVSFSVTRPEHNIAISW

SEQ ID NO: 77 - protein, 179 aa, Vibrio cholera
VEEALNIFDECRSPCSLTPEPGKPIQSKLSIPSDVVLDEGVLYYSMTINDEQNDIKDEDKGESIITIGEFATVRATRHYVNQDAPFGVIHLDITTENGTKTYSYNRKEGEFAINWLVPIGEDSPASIKISVDELDQQRNIIEVPKLYSIDLDNQTLEQWKTQGNVSFSVTRPEHNIAIS

SEQ ID NO: 78 - protein, 178 aa, Vibrio cholera
VEEALNIFDECRSPCSLTPEPGKPIQSKLSIPSDVVLDEGVLYYSMTINDEQNDIKDEDKGESIITIGEFATVRATRHYVNQDAPFGVIHLDITTENGTKTYSYNRKEGEFAINWLVPIGEDSPASIKISVDELDQQRNIIEVPKLYSIDLDNQTLEQWKTQGNVSFSVTRPEHNIAI

SEQ ID NO: 79 - protein, 177 aa, Vibrio cholera
VEEALNIFDECRSPCSLTPEPGKPIQSKLSIPSDVVLDEGVLYYSMTINDEQNDIKDEDKGESIITIGEFATVRATRHYVNQDAPFGVIHLDITTENGTKTYSYNRKEGEFAINWLVPIGEDSPASIKISVDELDQQRNIIEVPKLYSIDLDNQTLEQWKTQGNVSFSVTRPEHNIA

SEQ ID NO: 80 - protein, 176 aa, Vibrio cholera
VEEALNIFDECRSPCSLTPEPGKPIQSKLSIPSDVVLDEGVLYYSMTINDEQNDIKDEDKGESIITIGEFATVRATRHYVNQDAPFGVIHLDITTENGTKTYSYNRKEGEFAINWLVPIGEDSPASIKISVDELDQQRNIIEVPKLYSIDLDNQTLEQWKTQGNVSFSVTRPEHNI

SEQ ID NO: 81 - protein, 175 aa, Vibrio cholera
VEEALNIFDECRSPCSLTPEPGKPIQSKLSIPSDVVLDEGVLYYSMTINDEQNDIKDEDKGESIITIGEFATVRATRHYVNQDAPFGVIHLDITTENGTKTYSYNRKEGEFAINWLVPIGEDSPASIKISVDELDQQRNIIEVPKLYSIDLDNQTLEQWKTQGNVSFSVTRPEHN

SEQ ID NO: 82 - protein, 174 aa, Vibrio cholera
VEEALNIFDECRSPCSLTPEPGKPIQSKLSIPSDVVLDEGVLYYSMTINDEQNDIKDEDKGESIITIGEFATVRATRHYVNQDAPFGVIHLDITTENGTKTYSYNRKEGEFAINWLVPIGEDSPASIKISVDELDQQRNIIEVPKLYSIDLDNQTLEQWKTQGNVSFSVTRPEH

SEQ ID NO: 83 - protein, 173 aa, Vibrio cholera
VEEALNIFDECRSPCSLTPEPGKPIQSKLSIPSDVVLDEGVLYYSMTINDEQNDIKDEDKGESIITIGEFATVRATRHYVNQDAPFGVIHLDITTENGTKTYSYNRKEGEFAINWLVPIGEDSPASIKISVDELDQQRNIIEVPKLYSIDLDNQTLEQWKTQGNVSFSVTRPE

SEQ ID NO: 84 - protein, 172 aa, Vibrio cholera
VEEALNIFDECRSPCSLTPEPGKPIQSKLSIPSDVVLDEGVLYYSMTINDEQNDIKDEDKGESIITIGEFATVRATRHYVNQDAPFGVIHLDITTENGTKTYSYNRKEGEFAINWLVPIGEDSPASIKISVDELDQQRNIIEVPKLYSIDLDNQTLEQWKTQGNVSFSVTRP

SEQ ID NO: 85 - protein, 171 aa, Vibrio cholera
VEEALNIFDECRSPCSLTPEPGKPIQSKLSIPSDVVLDEGVLYYSMTINDEQNDIKDEDKGESIITIGEFATVRATRHYVNQDAPFGVIHLDITTENGTKTYSYNRKEGEFAINWLVPIGEDSPASIKISVDELDQQRNIIEVPKLYSIDLDNQTLEQWKTQGNVSFSVTR

SEQ ID NO: 86 - protein, 170 aa, Vibrio cholera
VEEALNIFDECRSPCSLTPEPGKPIQSKLSIPSDVVLDEGVLYYSMTINDEQNDIKDEDKGESIITIGEFATVRATRHYVNQDAPFGVIHLDITTENGTKTYSYNRKEGEFAINWLVPIGEDSPASIKISVDELDQQRNIIEVPKLYSIDLDNQTLEQWKTQGNVSFSVT

SEQ ID NO: 87 - protein, 169 aa, Vibrio cholera
VEEALNIFDECRSPCSLTPEPGKPIQSKLSIPSDVVLDEGVLYYSMTINDEQNDIKDEDKGESIITIGEFATVRATRHYVNQDAPFGVIHLDITTENGTKTYSYNRKEGEFAINWLVPIGEDSPASIKISVDELDQQRNIIEVPKLYSIDLDNQTLEQWKTQGNVSFSV

SEQ ID NO: 88 - protein, 168 aa, Vibrio cholera
VEEALNIFDECRSPCSLTPEPGKPIQSKLSIPSDVVLDEGVLYYSMTINDEQNDIKDEDKGESIITIGEFATVRATRHYVNQDAPFGVIHLDITTENGTKTYSYNRKEGEFAINWLVPIGEDSPASIKISVDELDQQRNIIEVPKLYSIDLDNQTLEQWKTQGNVSFS

SEQ ID NO: 89 - protein, 167 aa, Vibrio cholera
VEEALNIFDECRSPCSLTPEPGKPIQSKLSIPSDVVLDEGVLYYSMTINDEQNDIKDEDKGESIITIGEFATVRATRHYVNQDAPFGVIHLDITTENGTKTYSYNRKEGEFAINWLVPIGEDSPASIKISVDELDQQRNIIEVPKLYSIDLDNQTLEQWKTQGNVSF

SEQ ID NO: 90 - protein, 166 aa, Vibrio cholera
VEEALNIFDECRSPCSLTPEPGKPIQSKLSIPSDVVLDEGVLYYSMTINDEQNDIKDEDKGESIITIGEFATVRATRHYVNQDAPFGVIHLDITTENGTKTYSYNRKEGEFAINWLVPIGEDSPASIKISVDELDQQRNIIEVPKLYSIDLDNQTLEQWKTQGNVS

SEQ ID NO: 91 - protein, 165 aa, Vibrio cholera
VEEALNIFDECRSPCSLTPEPGKPIQSKLSIPSDVVLDEGVLYYSMTINDEQNDIKDEDKGESIITIGEFATVRATRHYVNQDAPFGVIHLDITTENGTKTYSYNRKEGEFAINWLVPIGEDSPASIKISVDELDQQRNIIEVPKLYSIDLDNQTLEQWKTQGNV

SEQ ID NO: 92 - protein, 164 aa, Vibrio cholera
VEEALNIFDECRSPCSLTPEPGKPIQSKLSIPSDVVLDEGVLYYSMTINDEQNDIKDEDKGESIITIGEFATVRATRHYVNQDAPFGVIHLDITTENGTKTYSYNRKEGEFAINWLVPIGEDSPASIKISVDELDQQRNIIEVPKLYSIDLDNQTLEQWKTQGN

SEQ ID NO: 93 - protein, 163 aa, Vibrio cholera
VEEALNIFDECRSPCSLTPEPGKPIQSKLSIPSDVVLDEGVLYYSMTINDEQNDIKDEDKGESIITIGEFATVRATRHYVNQDAPFGVIHLDITTENGTKTYSYNRKEGEFAINWLVPIGEDSPASIKISVDELDQQRNIIEVPKLYSIDLDNQTLEQWKTQG

SEQ ID NO: 94 - protein, 162 aa, Vibrio cholera
VEEALNIFDECRSPCSLTPEPGKPIQSKLSIPSDVVLDEGVLYYSMTINDEQNDIKDEDKGESIITIGEFATVRATRHYVNQDAPFGVIHLDITTENGTKTYSYNRKEGEFAINWLVPIGEDSPASIKISVDELDQQRNIIEVPKLYSIDLDNQTLEQWKTQ

SEQ ID NO: 95 - protein, 161 aa, Vibrio cholera
VEEALNIFDECRSPCSLTPEPGKPIQSKLSIPSDVVLDEGVLYYSMTINDEQNDIKDEDKGESIITIGEFATVRATRHYVNQDAPFGVIHLDITTENGTKTYSYNRKEGEFAINWLVPIGEDSPASIKISVDELDQQRNIIEVPKLYSIDLDNQTLEQWKT

SEQ ID NO: 96 - protein, 160 aa, Vibrio cholera
VEEALNIFDECRSPCSLTPEPGKPIQSKLSIPSDVVLDEGVLYYSMTINDEQNDIKDEDKGESIITIGEFATVRATRHYVNQDAPFGVIHLDITTENGTKTYSYNRKEGEFAINWLVPIGEDSPASIKISVDELDQQRNIIEVPKLYSIDLDNQTLEQWK

SEQ ID NO: 97 - protein, 159 aa, Vibrio cholera
VEEALNIFDECRSPCSLTPEPGKPIQSKLSIPSDVVLDEGVLYYSMTINDEQNDIKDEDKGESIITIGEFATVRATRHYVNQDAPFGVIHLDITTENGTKTYSYNRKEGEFAINWLVPIGEDSPASIKISVDELDQQRNIIEVPKLYSIDLDNQTLEQW

SEQ ID NO: 98 - protein, 158 aa, Vibrio cholera
VEEALNIFDECRSPCSLTPEPGKPIQSKLSIPSDVVLDEGVLYYSMTINDEQNDIKDEDKGESIITIGEFATVRATRHYVNQDAPFGVIHLDITTENGTKTYSYNRKEGEFAINWLVPIGEDSPASIKISVDELDQQRNIIEVPKLYSIDLDNQTLEQ

SEQ ID NO: 99 - protein, 157 aa, Vibrio cholera
VEEALNIFDECRSPCSLTPEPGKPIQSKLSIPSDVVLDEGVLYYSMTINDEQNDIKDEDKGESIITIGEFATVRATRHYVNQDAPFGVIHLDITTENGTKTYSYNRKEGEFAINWLVPIGEDSPASIKISVDELDQQRNIIEVPKLYSIDLDNQTLE

SEQ ID NO: 100 - protein, 156 aa, Vibrio cholera
VEEALNIFDECRSPCSLTPEPGKPIQSKLSIPSDVVLDEGVLYYSMTINDEQNDIKDEDKGESIITIGEFATVRATRHYVNQDAPFGVIHLDITTENGTKTYSYNRKEGEFAINWLVPIGEDSPASIKISVDELDQQRNIIEVPKLYSIDLDNQTL

SEQ ID NO: 101 - protein, 155 aa, Vibrio cholera
VEEALNIFDECRSPCSLTPEPGKPIQSKLSIPSDVVLDEGVLYYSMTINDEQNDIKDEDKGESIITIGEFATVRATRHYVNQDAPFGVIHLDITTENGTKTYSYNRKEGEFAINWLVPIGEDSPASIKISVDELDQQRNIIEVPKLYSIDLDNQT

SEQ ID NO: 102 - protein, 154 aa, Vibrio cholera
VEEALNIFDECRSPCSLTPEPGKPIQSKLSIPSDVVLDEGVLYYSMTINDEQNDIKDEDKGESIITIGEFATVRATRHYVNQDAPFGVIHLDITTENGTKTYSYNRKEGEFAINWLVPIGEDSPASIKISVDELDQQRNIIEVPKLYSIDLDNQ

SEQ ID NO: 103 - protein, 153 aa, Vibrio cholera
VEEALNIFDECRSPCSLTPEPGKPIQSKLSIPSDVVLDEGVLYYSMTINDEQNDIKDEDKGESIITIGEFATVRATRHYVNQDAPFGVIHLDITTENGTKTYSYNRKEGEFAINWLVPIGEDSPASIKISVDELDQQRNIIEVPKLYSIDLDN

SEQ ID NO: 104 - protein, 152 aa, Vibrio cholera
VEEALNIFDECRSPCSLTPEPGKPIQSKLSIPSDVVLDEGVLYYSMTINDEQNDIKDEDKGESIITIGEFATVRATRHYVNQDAPFGVIHLDITTENGTKTYSYNRKEGEFAINWLVPIGEDSPASIKISVDELDQQRNIIEVPKLYSIDLD

SEQ ID NO: 105 - protein, 151 aa, Vibrio cholera
VEEALNIFDECRSPCSLTPEPGKPIQSKLSIPSDVVLDEGVLYYSMTINDEQNDIKDEDKGESIITIGEFATVRATRHYVNQDAPFGVIHLDITTENGTKTYSYNRKEGEFAINWLVPIGEDSPASIKISVDELDQQRNIIEVPKLYSIDL

SEQ ID NO: 106 - protein, 150 aa, Vibrio cholera
VEEALNIFDECRSPCSLTPEPGKPIQSKLSIPSDVVLDEGVLYYSMTINDEQNDIKDEDKGESIITIGEFATVRATRHYVNQDAPFGVIHLDITTENGTKTYSYNRKEGEFAINWLVPIGEDSPASIKISVDELDQQRNIIEVPKLYSID

SEQ ID NO: 107 - protein, 151 aa, synthetic construct
  source 1..151: note = Description of Artificial Sequence: Synthetic polypeptide
MVEEALNIFDECRSPCSLTPEPGKPIQSKLSIPSDVVLDEGVLYYSMTINDEQNDIKDEDKGESIITIGEFATVRATRHYVNQDAPFGVIHLDITTENGTKTYSYNRKEGEFAINWLVPIGEDSPASIKISVDELDQQRNIIEVPKLYSID

SEQ ID NO: 108 - protein, 149 aa, Vibrio cholera
VEEALNIFDECRSPCSLTPEPGKPIQSKLSIPSDVVLDEGVLYYSMTINDEQNDIKDEDKGESIITIGEFATVRATRHYVNQDAPFGVIHLDITTENGTKTYSYNRKEGEFAINWLVPIGEDSPASIKISVDELDQQRNIIEVPKLYSI

SEQ ID NO: 109 - protein, 148 aa, Vibrio cholera
VEEALNIFDECRSPCSLTPEPGKPIQSKLSIPSDVVLDEGVLYYSMTINDEQNDIKDEDKGESIITIGEFATVRATRHYVNQDAPFGVIHLDITTENGTKTYSYNRKEGEFAINWLVPIGEDSPASIKISVDELDQQRNIIEVPKLYS

SEQ ID NO: 110 - protein, 147 aa, Vibrio cholera
VEEALNIFDECRSPCSLTPEPGKPIQSKLSIPSDVVLDEGVLYYSMTINDEQNDIKDEDKGESIITIGEFATVRATRHYVNQDAPFGVIHLDITTENGTKTYSYNRKEGEFAINWLVPIGEDSPASIKISVDELDQQRNIIEVPKLY

SEQ ID NO: 111 - protein, 146 aa, Vibrio cholera
VEEALNIFDECRSPCSLTPEPGKPIQSKLSIPSDVVLDEGVLYYSMTINDEQNDIKDEDKGESIITIGEFATVRATRHYVNQDAPFGVIHLDITTENGTKTYSYNRKEGEFAINWLVPIGEDSPASIKISVDELDQQRNIIEVPKL

SEQ ID NO: 112 - protein, 145 aa, Vibrio cholera
VEEALNIFDECRSPCSLTPEPGKPIQSKLSIPSDVVLDEGVLYYSMTINDEQNDIKDEDKGESIITIGEFATVRATRHYVNQDAPFGVIHLDITTENGTKTYSYNRKEGEFAINWLVPIGEDSPASIKISVDELDQQRNIIEVPK

SEQ ID NO: 113 - protein, 144 aa, Vibrio cholera
VEEALNIFDECRSPCSLTPEPGKPIQSKLSIPSDVVLDEGVLYYSMTINDEQNDIKDEDKGESIITIGEFATVRATRHYVNQDAPFGVIHLDITTENGTKTYSYNRKEGEFAINWLVPIGEDSPASIKISVDELDQQRNIIEVP

SEQ ID NO: 114 - protein, 143 aa, Vibrio cholera
VEEALNIFDECRSPCSLTPEPGKPIQSKLSIPSDVVLDEGVLYYSMTINDEQNDIKDEDKGESIITIGEFATVRATRHYVNQDAPFGVIHLDITTENGTKTYSYNRKEGEFAINWLVPIGEDSPASIKISVDELDQQRNIIEV

SEQ ID NO: 115 - protein, 142 aa, Vibrio cholera
VEEALNIFDECRSPCSLTPEPGKPIQSKLSIPSDVVLDEGVLYYSMTINDEQNDIKDEDKGESIITIGEFATVRATRHYVNQDAPFGVIHLDITTENGTKTYSYNRKEGEFAINWLVPIGEDSPASIKISVDELDQQRNIIE

SEQ ID NO: 116 - protein, 141 aa, Vibrio cholera
VEEALNIFDECRSPCSLTPEPGKPIQSKLSIPSDVVLDEGVLYYSMTINDEQNDIKDEDKGESIITIGEFATVRATRHYVNQDAPFGVIHLDITTENGTKTYSYNRKEGEFAINWLVPIGEDSPASIKISVDELDQQRNII

SEQ ID NO: 117 - protein, 140 aa, Vibrio cholera
VEEALNIFDECRSPCSLTPEPGKPIQSKLSIPSDVVLDEGVLYYSMTINDEQNDIKDEDKGESIITIGEFATVRATRHYVNQDAPFGVIHLDITTENGTKTYSYNRKEGEFAINWLVPIGEDSPASIKISVDELDQQRNI

SEQ ID NO: 118 - protein, 139 aa, Vibrio cholera
VEEALNIFDECRSPCSLTPEPGKPIQSKLSIPSDVVLDEGVLYYSMTINDEQNDIKDEDKGESIITIGEFATVRATRHYVNQDAPFGVIHLDITTENGTKTYSYNRKEGEFAINWLVPIGEDSPASIKISVDELDQQRN

SEQ ID NO: 119 - protein, 138 aa, Vibrio cholera
VEEALNIFDECRSPCSLTPEPGKPIQSKLSIPSDVVLDEGVLYYSMTINDEQNDIKDEDKGESIITIGEFATVRATRHYVNQDAPFGVIHLDITTENGTKTYSYNRKEGEFAINWLVPIGEDSPASIKISVDELDQQR

SEQ ID NO: 120 - protein, 137 aa, Vibrio cholera
VEEALNIFDECRSPCSLTPEPGKPIQSKLSIPSDVVLDEGVLYYSMTINDEQNDIKDEDKGESIITIGEFATVRATRHYVNQDAPFGVIHLDITTENGTKTYSYNRKEGEFAINWLVPIGEDSPASIKISVDELDQQ

SEQ ID NO: 121 - protein, 136 aa, Vibrio cholera
VEEALNIFDECRSPCSLTPEPGKPIQSKLSIPSDVVLDEGVLYYSMTINDEQNDIKDEDKGESIITIGEFATVRATRHYVNQDAPFGVIHLDITTENGTKTYSYNRKEGEFAINWLVPIGEDSPASIKISVDELDQ

SEQ ID NO: 122 - protein, 135 aa, Vibrio cholera
VEEALNIFDECRSPCSLTPEPGKPIQSKLSIPSDVVLDEGVLYYSMTINDEQNDIKDEDKGESIITIGEFATVRATRHYVNQDAPFGVIHLDITTENGTKTYSYNRKEGEFAINWLVPIGEDSPASIKISVDELD

SEQ ID NO: 123 - protein, 134 aa, Vibrio cholera
VEEALNIFDECRSPCSLTPEPGKPIQSKLSIPSDVVLDEGVLYYSMTINDEQNDIKDEDKGESIITIGEFATVRATRHYVNQDAPFGVIHLDITTENGTKTYSYNRKEGEFAINWLVPIGEDSPASIKISVDEL

SEQ ID NO: 124 - protein, 133 aa, Vibrio cholera
VEEALNIFDECRSPCSLTPEPGKPIQSKLSIPSDVVLDEGVLYYSMTINDEQNDIKDEDKGESIITIGEFATVRATRHYVNQDAPFGVIHLDITTENGTKTYSYNRKEGEFAINWLVPIGEDSPASIKISVDE

SEQ ID NO: 125 - protein, 134 aa, synthetic construct
  source 1..134: note = Description of Artificial Sequence: Synthetic polypeptide
MVEEALNIFDECRSPCSLTPEPGKPIQSKLSIPSDVVLDEGVLYYSMTINDEQNDIKDEDKGESIITIGEFATVRATRHYVNQDAPFGVIHLDITTENGTKTYSYNRKEGEFAINWLVPIGEDSPASIKISVDE

SEQ ID NO: 126 - protein, 121 aa, Vibrio cholera
GNAMSALAAHRVCGVPLETLARSRKPRDLTDDLSCAYQAQNIVSLFVATRILFSHLDSVFTLNLDEQEPEVAERLSDLRRINENNPGMVTQVLTVARQIYNDYVTHHPGLTPEQTSAGAQA

SEQ ID NO: 127 - protein, 39 aa, Vibrio cholera
ADILSLFCPDADKSCVASNNDQANINIESRSGRSYLPEN

SEQ ID NO: 128 - protein, 209 aa, Vibrio cholera
RAVITPQGVTNWTYQELEATHQALTREGYVFVGYHGTNHVAAQTIVNRIAPVPRGNNTENEEKWGGLYVATHAEVAHGYARIKEGTGEYGLPTRAERDARGVMLRVYIPRASLERFYRTNTPLENAEEHITQVIGHSLPLRNEAFTGPESAGGEDETVIGWDMAIHAVAIPSTIPGNAYEELAIDEEAVAKEQSISTKPPYKERKDELK

SEQ ID NO: 129 - protein, 425 aa, Vibrio cholera
VEEALNIFDECRSPCSLTPEPGKPIQSKLSIPSDVVLDEGVLYYSMTINDEQNDIKDEDKGESIITIGEFATVRATRHYVNQDAPFGVIHLDITTENGTKTYSYNRKEGEFAINWLVPIGEDSPASIKISVDELDQQRNIIEVPKLYSIDLDNQTLEQWKTQGNVSFSVTRPEHNIAISWPSVSYKAAQKEGSRHKRWAHWHTGLALCWLVPMDAIYNYITQQNCTLGDNWFGGSYETVAGTPKVITVKQGIEQKPVEQRIHFSKGNAMSALAAHRVCGVPLETLARSRKPRDLTDDLSCAYQAQNIVSLFVATRILFSHLDSVFTLNLDEQEPEVAERLSDLRRINENNPGMVTQVLTVARQIYNDYVTHHPGLTPEQTSAGAQAADILSLFCPDADKSCVASNNDQANINIESRSGRSYLPEN

SEQ ID NO: 130 - protein, 415 aa, Vibrio cholera
VEEALNIFDECRSPCSLTPEPGKPIQSKLSIPSDVVLDEGVLYYSMTINDEQNDIKDEDKGESIITIGEFATVRATRHYVNQDAPFGVIHLDITTENGTKTYSYNRKEGEFAINWLVPIGEDSPASIKISVDELDQQRNIIEVPKLYSIDLDNQTLEQWKTQGNVSFSVTRPEHNIAISWPSVSYKAAQKEGSRHKRWAHWHTGLALCWLVPMDAIYNYITQQNCTLGDNWFGGSYETVAGTPKVITVKQGIEQKPVEQRIHFSKGNAMSALAAHRVCGVPLETLARSRKPRDLTDDLSCAYQAQNIVSLFVATRILFSHLDSVFTLNLDEQEPEVAERLSDLRRINENNPGMVTQVLTVARQIYNDYVTHHPGLTPEQTSAGAQAADILSLFCPDADKSCVASNNDQANINIES

SEQ ID NO: 131 - protein, 397 aa, Vibrio cholera
VEEALNIFDECRSPCSLTPEPGKPIQSKLSIPSDVVLDEGVLYYSMTINDEQNDIKDEDKGESIITIGEFATVRATRHYVNQDAPFGVIHLDITTENGTKTYSYNRKEGEFAINWLVPIGEDSPASIKISVDELDQQRNIIEVPKLYSIDLDNQTLEQWKTQGNVSFSVTRPEHNIAISWPSVSYKAAQKEGSRHKRWAHWHTGLALCWLVPMDAIYNYITQQNCTLGDNWFGGSYETVAGTPKVITVKQGIEQKPVEQRIHFSKGNAMSALAAHRVCGVPLETLARSRKPRDLTDDLSCAYQAQNIVSLFVATRILFSHLDSVFTLNLDEQEPEVAERLSDLRRINENNPGMVTQVLTVARQIYNDYVTHHPGLTPEQTSAGAQAADILSLFCPDA

SEQ ID NO: 132 - protein, 386 aa, Vibrio cholera
VEEALNIFDECRSPCSLTPEPGKPIQSKLSIPSDVVLDEGVLYYSMTINDEQNDIKDEDKGESIITIGEFATVRATRHYVNQDAPFGVIHLDITTENGTKTYSYNRKEGEFAINWLVPIGEDSPASIKISVDELDQQRNIIEVPKLYSIDLDNQTLEQWKTQGNVSFSVTRPEHNIAISWPSVSYKAAQKEGSRHKRWAHWHTGLALCWLVPMDAIYNYITQQNCTLGDNWFGGSYETVAGTPKVITVKQGIEQKPVEQRIHFSKGNAMSALAAHRVCGVPLETLARSRKPRDLTDDLSCAYQAQNIVSLFVATRILFSHLDSVFTLNLDEQEPEVAERLSDLRRINENNPGMVTQVLTVARQIYNDYVTHHPGLTPEQTSAGAQA

SEQ ID NO: 133 - protein, 291 aa, Vibrio cholera
VEEALNIFDECRSPCSLTPEPGKPIQSKLSIPSDVVLDEGVLYYSMTINDEQNDIKDEDKGESIITIGEFATVRATRHYVNQDAPFGVIHLDITTENGTKTYSYNRKEGEFAINWLVPIGEDSPASIKISVDELDQQRNIIEVPKLYSIDLDNQTLEQWKTQGNVSFSVTRPEHNIAISWPSVSYKAAQKEGSRHKRWAHWHTGLALCWLVPMDAIYNYITQQNCTLGDNWFGGSYETVAGTPKVITVKQGIEQKPVEQRIHFSKGNAMSALAAHRVCGVPLETLARSRKP

SEQ ID NO: 134 - DNA, 1902 bp, Vibrio cholera
  source 1..1902: mol_type = genomic DNA
gtcgaagaagctttaaacatctttgatgaatgccgttcgccatgttcgttgaccccggaaccgggtaagccgattcaatcaaaactgtctatccctagtgatgttgttctggatgaaggtgttctgtattactcgatgacgattaatgatgagcagaatgatattaaggatgaggacaaaggcgagtccattatcactattggtgaatttgccacagtacgcgcgactagacattatgttaatcaagatgcgccttttggtgtcatccatttagatattacgacagaaaatggtacaaaaacgtactcttataaccgcaaagagggtgaatttgcaatcaattggttagtgcctattggtgaagattctcctgcaagcatcaaaatctccgttgatgagctcgatcagcaacgcaatatcatcgaggtgcctaaactgtatagtattgatctcgataaccaaacgttagagcagtggaaaacccaaggtaatgtttctttttcggtaacgcgtcctgaacataatatcgctatctcttggccaagcgtgagttacaaagcagcgcagaaagagggttcacgccataagcgttgggctcattggcatacaggcttagcactgtgttggcttgtgccaatggatgctatctataactatatcacccagcaaaattgtactttaggggataattggtttggtggctcttatgagactgttgcaggcactccgaaggtgattacggttaagcaagggattgaacaaaagccagttgagcagcgcatccatttctccaaggggaatgcgatgagcgcacttgctgctcatcgcgtctgtggtgtgccattagaaactttggcgcgcagtcgcaaacctcgtgatctgacggatgatttatcatgtgcctatcaagcgcagaatatcgtgagtttatttgtcgcgacgcgtatcctgttctctcatctggatagcgtatttactctgaatcttgacgaacaagaaccagaggtggctgaacgtctaagtgatcttcgccgtatcaatgaaaataacccgggcatggttacacaggttttaaccgttgctcgtcagatctataacgattatgtcactcaccatccgggcttaactcctgagcaaaccagtgcgggtgcacaagctgccgatatcctctctttattttgcccagatgctgataagtcttgtgtggcttcaaacaacgatcaagccaatatcaacatcgagtctcgttctggccgttcatatttgcctgaaaaccgtgcggtaatcacccctcaaggcgtcacaaattggacttaccaggaactcgaagcaacacatcaagctctgactcgtgagggttatgtgttcgtgggttaccatggtacgaatcatgtcgctgcgcaaaccatcgtgaatcgcattgcccctgttccgcgcggcaacaacactgaaaacgaggaaaagtggggcgggttatatgttgcaactcacgctgaagttgcccatggttatgctcgcatcaaagaagggacaggggagtatggccttccgacccgtgctgagcgcgacgctcgtggggtaatgctgcgcgtgtatatccctcgtgcttcattagaacgtttttatcgcacgaatacacctttggaaaatgctgaggagcatatcacgcaagtgattggtcattctttgccattacgcaatgaagcatttactggtccagaaagtgcgggcggggaagacgaaactgtcattggctgggatatggcgattcatgcagttgcgatcccttcgactatcccagggaacgcttacgaagaattggcgattgatgaggaggctgttgcaaaagagcaatcgattagcacaaaaccaccttataaagagcgcaaagatgaacttaag

SEQ ID NO: 135 - protein, 613 aa, Pseudomonas aeruginosa
AEEAFDLWNECAKACVLDLKDGVRSSRMSVDPAIADTNGQGVLHYSMVLEGGNDALKLAIDNALSITSDGLTIRLEGGVEPNKPVRYSYTRQARGSWSLNWLVPIGHEKPSNIKVFIHELNAGNQLSHMSPIYTIEMGDELLAKLARDATFFVRAHESNEMQPTLAISHAGVSVVMAQAQPRREKRWSEWASGKVLCLLDPLDGVYNYLAQQRCNLDDTWEGKIYRVLAGNPAKHDLDIKPTVISHRLHFPEGGSLAALTAHQACHLPLETFTRHRQPRGWEQLEQCGYPVQRLVALYLAARLSWNQVDQVIRNALASPGSGGDLGEAIREQPEQARLALTLAAAESERFVRQGTGNDEAGAASADVVSLTCPVAAGECAGPADSGDALLERNYPTGAEFLGDGGDVSFSTRGTQNWTVERLLQAHRQLEERGYVFVGYHGTFLEAAQSIVFGGVRARSQDLDAIWRGFYIAGDPALAYGYAQDQEPDARGRIRNGALLRVYVPRSSLPGFYRTGLTLAAPEAAGEVERLIGHPLPLRLDAITGPEEEGGRLETILGWPLAERTVVIPSAIPTDPRNVGGDLDPSSIPDKEQAISALPDYASQPGKPPREDLK

SEQ ID NO: 136 - DNA, 1839 bp, Pseudomonas aeruginosa
  source 1..1839: mol_type = genomic DNA
gccgaggaagccttcgacctctggaacgaatgcgccaaggcctgcgtgctcgacctcaaggacggcgtgcgttccagccgcatgagcgtcgacccggccatcgccgacaccaacggccagggcgtgctgcactactccatggtcctggagggcggcaacgacgcgctcaagctggccatcgacaacgccctcagcatcaccagcgacggcctgaccatccgcctcgaaggtggcgtcgagccgaacaagccggtgcgctacagctacacgcgccaggcgcgcggcagttggtcgctgaactggctggtgccgatcggccacgagaagccttcgaacatcaaggtgttcatccacgaactgaacgccggtaaccagctcagccacatgtcgccgatctacaccatcgagatgggcgacgagttgctggcgaagctggcgcgcgatgccaccttcttcgtcagggcgcacgagagcaacgagatgcagccgacgctcgccatcagccatgccggggtcagcgtggtcatggcccaggcccagccgcgccgggaaaagcgctggagcgaatgggccagcggcaaggtgttgtgcctgctcgacccgctggacggggtctacaactacctcgcccagcagcgctgcaacctcgacgatacctgggaaggcaagatctaccgggtgctcgccggcaacccggcgaagcatgacctggacatcaagcccacggtcatcagtcatcgcctgcatttccccgagggcggcagcctggccgcgctgaccgcgcaccaggcctgccacctgccgctggagaccttcacccgtcatcgccagccgcgcggctgggaacaactggagcagtgcggctatccggtgcagcggctggtcgccctctacctggcggcgcggctgtcgtggaaccaggtcgaccaggtgatccgcaacgccctggccagccccggcagcggcggcgacctgggcgaagcgatccgcgagcagccggagcaggcccgtctggccctgaccctggccgccgccgagagcgagcgcttcgtccggcagggcacaggcaacgacgaggccggcgcggccagcgccgacgtggtgagcctgacctgcccggtcgccgccggtgaatgcgcgggcccggcggacagcggcgacgccctgctggagcgcaactatcccactggcgcggagttcctcggcgacggcggcgacatcagcttcagcacccgcggcacgcagaactggacggtggagcggctgctccaggcgcaccgccaactggaggagcgcggctatgtgttcgtcggctaccacggcaccttcctcgaagcggcgcaaagcatcgtcttcggcggggtgcgcgcgcgcagccaggacctcgacgcgatctggcgcggtttctatatcgccggcgatccggcgctggcctacggctacgcccaggaccaggaacccgacgcgcgcggccggatccgcaacggtgccctgctgcgggtctatgtgccgcgctcgagtctgccgggcttctaccgcaccggcctgaccctggccgcgccggaggcggcgggcgaggtcgaacggctgatcggccatccgctgccgctgcgcctggacgccatcaccggccccgaggaggaaggcgggcgcctggaaaccattctcggctggccgctggccgagcgcaccgtggtgattccctcggcgatccccaccgacccgcgcaacgtcggcggcgacctcgacccgtccagcatccccgacaaggaacaggcgatcagcgccctgccggactacgccagccagcccggcaaaccgccgcgcgaggacctgaag

SEQ ID NO: 137 - protein, 252 aa, Pseudomonas aeruginosa
AEEAFDLWNECAKACVLDLKDGVRSSRMSVDPAIADTNGQGVLHYSMVLEGGNDALKLAIDNALSITSDGLTIRLEGGVEPNKPVRYSYTRQARGSWSLNWLVPIGHEKPSNIKVFIHELNAGNQLSHMSPIYTIEMGDELLAKLARDATFFVRAHESNEMQPTLAISHAGVSVVMAQAQPRREKRWSEWASGKVLCLLDPLDGVYNYLAQQRCNLDDTWEGKIYRVLAGNPAKHDLDIKPTVISHRLHFPE

SEQ ID NO: 138 - protein, 112 aa, Pseudomonas aeruginosa
GGSLAALTAHQACHLPLETFTRHRQPRGWEQLEQCGYPVQRLVALYLAARLSWNQVDQVIRNALASPGSGGDLGEAIREQPEQARLALTLAAAESERFVRQGTGNDEAGAAS

SEQ ID NO: 139 - protein, 40 aa, Pseudomonas aeruginosa
ADVVSLTCPVAAGECAGPADSGDALLERNYPTGAEFLGDG

SEQ ID NO: 140 - protein, 209 aa, Pseudomonas aeruginosa
GDVSFSTRGTQNWTVERLLQAHRQLEERGYVFVGYHGTFLEAAQSIVFGGVRARSQDLDAIWRGFYIAGDPALAYGYAQDQEPDARGRIRNGALLRVYVPRSSLPGFYRTGLTLAAPEAAGEVERLIGHPLPLRLDAITGPEEEGGRLETILGWPLAERTVVIPSAIPTDPRNVGGDLDPSSIPDKEQAISALPDYASQPGKPPREDLK

SEQ ID NO: 141 - protein, 404 aa, Pseudomonas aeruginosa
AEEAFDLWNECAKACVLDLKDGVRSSRMSVDPAIADTNGQGVLHYSMVLEGGNDALKLAIDNALSITSDGLTIRLEGGVEPNKPVRYSYTRQARGSWSLNWLVPIGHEKPSNIKVFIHELNAGNQLSHMSPIYTIEMGDELLAKLARDATFFVRAHESNEMQPTLAISHAGVSVVMAQAQPRREKRWSEWASGKVLCLLDPLDGVYNYLAQQRCNLDDTWEGKIYRVLAGNPAKHDLDIKPTVISHRLHFPEGGSLAALTAHQACHLPLETFTRHRQPRGWEQLEQCGYPVQRLVALYLAARLSWNQVDQVIRNALASPGSGGDLGEAIREQPEQARLALTLAAAESERFVRQGTGNDEAGAASADVVSLTCPVAAGECAGPADSGDALLERNYPTGAEFLGDG

SEQ ID NO: 142 - protein, 395 aa, Pseudomonas aeruginosa
AEEAFDLWNECAKACVLDLKDGVRSSRMSVDPAIADTNGQGVLHYSMVLEGGNDALKLAIDNALSITSDGLTIRLEGGVEPNKPVRYSYTRQARGSWSLNWLVPIGHEKPSNIKVFIHELNAGNQLSHMSPIYTIEMGDELLAKLARDATFFVRAHESNEMQPTLAISHAGVSVVMAQAQPRREKRWSEWASGKVLCLLDPLDGVYNYLAQQRCNLDDTWEGKIYRVLAGNPAKHDLDIKPTVISHRLHFPEGGSLAALTAHQACHLPLETFTRHRQPRGWEQLEQCGYPVQRLVALYLAARLSWNQVDQVIRNALASPGSGGDLGEAIREQPEQARLALTLAAAESERFVRQGTGNDEAGAASADVVSLTCPVAAGECAGPADSGDALLERNYP

SEQ ID NO: 143 - protein, 375 aa, Pseudomonas aeruginosa
AEEAFDLWNECAKACVLDLKDGVRSSRMSVDPAIADTNGQGVLHYSMVLEGGNDALKLAIDNALSITSDGLTIRLEGGVEPNKPVRYSYTRQARGSWSLNWLVPIGHEKPSNIKVFIHELNAGNQLSHMSPIYTIEMGDELLAKLARDATFFVRAHESNEMQPTLAISHAGVSVVMAQAQPRREKRWSEWASGKVLCLLDPLDGVYNYLAQQRCNLDDTWEGKIYRVLAGNPAKHDLDIKPTVISHRLHFPEGGSLAALTAHQACHLPLETFTRHRQPRGWEQLEQCGYPVQRLVALYLAARLSWNQVDQVIRNALASPGSGGDLGEAIREQPEQARLALTLAAAESERFVRQGTGNDEAGAASADVVSLTCPVA

SEQ ID NO: 144 - protein, 364 aa, Pseudomonas aeruginosa
AEEAFDLWNECAKACVLDLKDGVRSSRMSVDPAIADTNGQGVLHYSMVLEGGNDALKLAIDNALSITSDGLTIRLEGGVEPNKPVRYSYTRQARGSWSLNWLVPIGHEKPSNIKVFIHELNAGNQLSHMSPIYTIEMGDELLAKLARDATFFVRAHESNEMQPTLAISHAGVSVVMAQAQPRREKRWSEWASGKVLCLLDPLDGVYNYLAQQRCNLDDTWEGKIYRVLAGNPAKHDLDIKPTVISHRLHFPEGGSLAALTAHQACHLPLETFTRHRQPRGWEQLEQCGYPVQRLVALYLAARLSWNQVDQVIRNALASPGSGGDLGEAIREQPEQARLALTLAAAESERFVRQGTGNDEAGAAS

SEQ ID NO: 145 - protein, 277 aa, Pseudomonas aeruginosa
AEEAFDLWNECAKACVLDLKDGVRSSRMSVDPAIADTNGQGVLHYSMVLEGGNDALKLAIDNALSITSDGLTIRLEGGVEPNKPVRYSYTRQARGSWSLNWLVPIGHEKPSNIKVFIHELNAGNQLSHMSPIYTIEMGDELLAKLARDATFFVRAHESNEMQPTLAISHAGVSVVMAQAQPRREKRWSEWASGKVLCLLDPLDGVYNYLAQQRCNLDDTWEGKIYRVLAGNPAKHDLDIKPTVISHRLHFPEGGSLAALTAHQACHLPLETFTRHRQ

SEQ ID NO: 146 - protein, 627 aa, synthetic construct
  source 1..627: note = Description of Artificial Sequence: Synthetic polypeptide
MVEEALNIFDECRSPCSLTPEPGKPIQSKLSIPSDVVLDEGVLYYSMTINDEQNDIKDEDKGESIITIGEFATVRATRHYVNQDAPFGVIHLDITTENGTKTYSYNRKEGEFAINWLVPIGEDSPASIKISVDELDQQRNIIEVPKLYSIDLDNQTLEQWKTQGNVSFSVTRPEHNIAISWPSVSYKAAQKEGSRHKRWAHWHTGLALCWLVPMDAIYNYITQQNCTLGDNWFGGSYETVAGTPKVITVKQGIEQKPVEQRIHFSKGGGSLAALTAHQACHLPLETFTRHRQPRGWEQLEQCGYPVQRLVALYLAARLSWNQVDQVIRNALASPGSGGDLGEAIREQPEQARLALTLAAAESERFVRQGTGNDEAGAASADVVSLTCPVAAGECAGPADSGDALLERNYPTGAEFLGDGGDVSFSTRGTQNWTVERLLQAHRQLEERGYVFVGYHGTFLEAAQSIVFGGVRARSQDLDAIWRGFYIAGDPALAYGYAQDQEPDARGRIRNGALLRVYVPRSSLPGFYRTSLTLAAPEAAGEVERLIGHPLPLRLDAITGPEEEGGRLTILGWPLAERTVVIPSAIPTDPRNVGGDLDPSSIPDKEQAISALPDYASQPGKPPREDLK

SEQ ID NO: 147 - protein, 620 aa, synthetic construct
  source 1..620: note = Description of Artificial Sequence: Synthetic polypeptide
MAEEAFDLWNECAKACVLDLKDGVRSSRMSVDPAIADTNGQGVLHYSMVLEGGNDALKLAIDNALSITSDGLTIRLEGGVEPNKPVRYSYTRQARGSWSLNWLVPIGHEKPSNIKVFIHELNAGNQLSHMSPIYTIEMGDELLAKLARDATFFVRAHESNEMQPTLAISHAGVSVVMAQTQPRREKRWSEWASGKVLCLLDPLDGVYNYLAQQRCNLDDTWEGKIYRVLAGNPAKHDLDIKPTVISHRLHFPEGGNAMSALAAHRVCGVPLETLARSRKPRDLTDDLSCAYQAQNIVSLFVATRILFSHLDSVFTLNLDEQEPEVAERLSDLRRINENNPGMVTQVLTVARQIYNDYVTHHPGLTPEQTSAGAQAAEILSLFCPDADKSCVATNNDQANINIESRSGRSYLPENRAVITPQGVTNWTYQELEATHQALTREGYVFVGYTNHVAAQTIVNRIAPVPRGNNTENEEKWGGLYVATHAEVAHGYARIKEGTGEYGLPTRAERDARGVMLRVYIPRASLERFYRTNTPLENAEEHITQVIGHSLPLRNEAFTGPESAGGEDTVIGWDMAIHAVAIPSTIPGNAYEELAIDEEAVAKEQSISTKPPYKERKDELK

SEQ ID NO: 148 - protein, 18 aa, Vibrio cholera
ELDQQRNIIEVPKLYSID

SEQ ID NO: 149 - protein, 39 aa, synthetic construct
  source 1..39: note = Description of Artificial Sequence: Synthetic polypeptide
MVEEALNIFDECRSPCSLTPEPGKPIQSKLSIPSDVVLD

SEQ ID NO: 150 - protein, 38 aa, Vibrio cholera
VEEALNIFDECRSPCSLTPEPGKPIQSKLSIPSDVVLD

SEQ ID NO: 151 - protein, 37 aa, Vibrio cholera
DLDNQTLEQWKTQGNVSFSVTRPEHNIAISWPSVSYK

SEQ ID NO: 152 - protein, 22 aa, Vibrio cholera
KAAQKEGSRHKRWAHWHTGLAL

SEQ ID NO: 153 - protein, 593 aa, synthetic construct
  source 1..593: note = Description of Artificial Sequence: Synthetic polypeptide
MVEEALNIFDECRSPCSLTPEPGKPIQSKLSIPSDVVLDEGVLYYSMTINDEQNDIKDEDKGESIITIGEFATVRATRHYVNQDAPFGVIHLDITTENGTKTYSYNRKEGEFAINWLVPIGEDSPASIKISVDELDQQRNIIEVPKLYSIDLDNQTLEQWKTQGNVSFSVTRPEHNIAISWPSVSYKAAQKEGSRHKRWAHWHTGLALCWLVPMDAIYNYITQQNCTLGDNWFGGSYETVAGTPKVITVKQGIEQKPVEQRIHFSKGNAMSALAAHRVCGVPLETLARSRKPRDLTDDLSCAYQAQNIVSLFVATRILFSHLDSVFTLNLDEQEPEVAERLSDLRRINENNPGMVTQVLTVARQIYNDYVTHHPGLTPEQTSAGAQAGGGGSGGGGSGGGGSFPTIPLSRLFDNAMLRAHRLHQLAFDTYQEFEEAYIPKEQKYSFLQNPQTSLCFSESIPTPSNREETQQKSNLELLRISLLLIQSWLEPVQFLRSVFANSLVYGASDSNVYDLLKDLEEGIQTLMGRLEDGSPRTGQIFKQTYSKFDTNSHNDDALLKNYGLLYCFRKDMDKVETFLRIVQCRSVEGSCGF

SEQ ID NO: 154 - protein, 580 aa, synthetic construct
  source 1..580: note = Description of Artificial Sequence: Synthetic polypeptide
MVEEALNIFDECRSPCSLTPEPGKPIQSKLSIPSDVVLDEGVLYYSMTINDEQNDIKDEDKGESIITIGEFATVRATRHYVNQDAPFGVIHLDITTENGTKTYSYNRKEGEFAINWLVPIGEDSPASIKISVDELDQQRNIIEVPKLYSIDLDNQTLEQWKTQGNVSFSVTRPEHNIAISWPSVSYKAAQKEGSRHKRWAHWHTGLALCWLVPMDAIYNYITQQNCTLGDNWFGGSYETVAGTPKVITVKQGIEQKPVEQRIHFSKGNAMSALAAHRVCGVPLETLARSRKPRDLTDDLSCAYQAQNIVSLFVATRILFSHLDSVFTLNLDEQEPEVAERLSDLRRINENNPGMVTQVLTVARQIYNDYVTHHPGLTPEQTSAGAQAGGGGSGGGGSGGGGSMHSSALLCCLVLLTGVRASPGQGTQSENSCTHFPGNLPNMLRDLRDAFSRVKTFFQMKDQLDNLLLKESLLEDFKGYLGCQALSEMIQFYLEEVMPQAENQDPDIKAHVNSLGENLKTLRLRLRRCHRFLPCENKSKAVEQVKNAFNKLQEKGIYKAMSEFDIFINYIEAYMTMKIRN

SEQ ID NO: 155 - protein, 460 aa, synthetic construct
  source 1..460: note = Description of Artificial Sequence: Synthetic polypeptide
MVEEALNIFDECRSPCSLTPEPGKPIQSKLSIPSDVVLDEGVLYYSMTINDEQNDIKDEDKGESIITIGEFATVRATRHYVNQDAPFGVIHLDITTENGTKTYSYNRKEGEFAINWLVPIGEDSPASIKISVDELDQQRNIIEVPKLYSIDLDNQTLEQWKTQGNVSFSVTRPEHNIAISWPSVSYKAAQKEGSRHKRWAHWHTGLALCWLVPMDAIYNYITQQNCTLGDNWFGGSYETVAGTPKVITVKQGIEQKPVEQRIHFSKGGGGSGGGGSGGGGSMAALQKSVSSFLMGTLATSCLLLLALLVQGGAAAPISSHCRLDKSNFQQPYITNRTFMLAKEASLADNNTDVRLIGEKLFHGVSMSERCYLMKQVLNFTLEEVLFPQSDRFQPYMQEVVPFLARLSNRLSTCHIEGDDLHIQRNVQKLKDTVKKLGESGEIKAIGELDLLFMSLRNACI

SEQ ID NO: 156 - protein, 491 aa, synthetic construct
  source 1..491: note = Description of Artificial Sequence: Synthetic polypeptide
MVEEALNIFDECRSPCSLTPEPGKPIQSKLSIPSDVVLDEGVLYYSMTINDEQNDIKDEDKGESIITIGEFATVRATRHYVNQDAPFGVIHLDITTENGTKTYSYNRKEGEFAINWLVPIGEDSPASIKISVDELDQQRNIIEVPKLYSIDLDNQTLEQWKTQGNVSFSVTRPEHNIAISWPSVSYKAAQKEGSRHKRWAHWHTGLALCWLVPMDAIYNYITQQNCTLGDNWFGGSYETVAGTPKVITVKQGIEQKPVEQRIHFSKMRSSKNVIKEFMRFKVRMEGTVNGHEFEIEGEGEGRPYEGHNTVKLKVTKGGPLPFAWDILSPQFQYGSKVYVKHPADIPDYKKLSFPEGFKWERVMNFEDGGVVTVTQDSSLQDGCFIYKVKFIGVNFPSDGPVMQKKTMGWEASTERLYPRDGVLKGEIHKALKLKDGGHYLVEFKSIYMAKKPVQLPGYYYVDSKLDITSHNEDYTIVEQYERTEGRHHLFL

SEQ ID NO: 157 - protein, 859 aa, synthetic construct
  source 1..859: note = Description of Artificial Sequence: Synthetic polypeptide
VEDELNIFDECRSPCSLTPEPGKPIQSKLSIPSDVVLDEGVLYYSMTINDEQNDIKDEDKGESIITIGEFATVRATRHYVNQDAPFGVIHLDITTENGTKTYSYNRKEGEFAINWLVPIGEDSPASIKISVDELDQQRNIIEVPKLYSIDLDNQTLEQWKTQGNVSFSVTRPEHNIAISWPSVSYKAAQKEGSRHKRWAHWHTGLALCWLVPMDAIYNYITQQNCTLGDNWFGGSYETVAGTPKVITVKQGIEQKPVEQRIHFSKGNAMSALAAHRVCGVPLETLARSRKPRDLTDDLSCAYQAQNIVSLFVATRILFSHLDSVFTLNLDEQEPEVAERLSDLRRINENNPGMVTQVLTVARQIYNDYVTHHPGLTPEQTSAGAQAADILSLFCPDADKSCVASNNDQANINIESRSGRSYLPENRAVITPQGVTNWTYQELEATHQALTREGYVFVGYHGTNHVAAQTIVNRIAPVPRGNNTENEEKWGGLYVATHAEVAHGYARIKEGTGEYGLPTRAERDARGVMLRVYIPRASLERFYRTNTPLENAEEHITQVIGHSLPLRNEAFTGPESAGGEDATVIGWDMAIHAVAIPSTIPGNAYEELAIDEEAVAKEQSISTKPPYKERKDELKMRSSKNVIKEFMRFKVRMEGTVNGHEFEIEGEGEGRPYEGHNTVKLKVTKGGPLPFAWDILSPQFQYGSKVYVKHPADIPDYKKLSFPEGFKWERVMNFEDGGVVTVTQDSSLQDGCFIYKVKFIGVNFPSDGPVMQKKTMGWEASTERLYPRDGVLKGEIHKALKLKDGGHYLVEFKSIYMAKKPVQLPGYYYVDSKLDITSHNEDYTIVEQYERTEGRHHLFL

SEQ ID NO: 158 - protein, 340 aa, synthetic construct
  source 1..340: note = Description of Artificial Sequence: Synthetic polypeptide
MVEEALNIFDECRSPCSLTPEPGKPIQSKLSIPSDVVLDEGVLYYSMTINDEQNDIKDEDKGESIITIGEFATVRATRHYVNQDAPFGVIHLDITTENGTKTYSYNRKEGEFAINWLVPIGEDSPASIKISVDEGGGGSGGGGSGGGGSFPTIPLSRLFDNAMLRAHRLHQLAFDTYQEFEEAYIPKEQKYSFLQNPQTSLCFSESIPTPSNREETQQKSNLELLRISLLLIQSWLEPVQFLRSVFANSLVYGASDSNVYDLLKDLEEGIQTLMGRLEDGSPRTGQIFKQTYSKFDTNSHNDDALLKNYGLLYCFRKDMDKVETFLRIVQCRSVEGSCGF

SEQ ID NO: 159 - protein, 357 aa, synthetic construct
  source 1..357: note = Description of Artificial Sequence: Synthetic polypeptide
MVEEALNIFDECRSPCSLTPEPGKPIQSKLSIPSDVVLDEGVLYYSMTINDEQNDIKDEDKGESIITIGEFATVRATRHYVNQDAPFGVIHLDITTENGTKTYSYNRKEGEFAINWLVPIGEDSPASIKISVDELDQQRNIIEVPKLYSIDGGGGSGGGGSGGGGSFPTIPLSRLFDNAMLRAHRLHQLAFDTYQEFEEAYIPKEQKYSFLQNPQTSLCFSESIPTPSNREETQQKSNLELLRISLLLIQSWLEPVQFLRSVFANSLVYGASDSNVYDLLKDLEEGIQTLMGRLEDGSPRTGQIFKQTYSKFDTNSHNDDALLKNYGLLYCFRKDMDKVETFLRIVQCRSVEGSCGF

SEQ ID NO: 160 - protein, 393 aa, synthetic construct
  source 1..393: note = Description of Artificial Sequence: Synthetic polypeptide
MVEEALNIFDECRSPCSLTPEPGKPIQSKLSIPSDVVLDEGVLYYSMTINDEQNDIKDEDKGESIITIGEFATVRATRHYVNQDAPFGVIHLDITTENGTKTYSYNRKEGEFAINWLVPIGEDSPASIKISVDELDQQRNIIEVPKLYSIDLDNQTLEQWKTQGNVSFSVTRPEHNIAISWPSVSYKGGGGSGGGGSGGGGSFPTIPLSRLFDNAMLRAHRLHQLAFDTYQEFEEAYIPKEQKYSFLQNPQTSLCFSESIPTPSNREETQQKSNLELLRISLLLIQSWLEPVQFLRSVFANSLVYGASDSNVYDLLKDLEEGIQTLMGRLEDGSPRTGQIFKQTYSKFDTNSHNDDALLKNYGLLYCFRKDMDKVETFLRIVQCRSVEGSCGF

SEQ ID NO: 161 - protein, 412 aa, synthetic construct
  source 1..412: note = Description of Artificial Sequence: Synthetic polypeptide
MVEEALNIFDECRSPCSLTPEPGKPIQSKLSIPSDVVLDEGVLYYSMTINDEQNDIKDEDKGESIITIGEFATVRATRHYVNQDAPFGVIHLDITTENGTKTYSYNRKEGEFAINWLVPIGEDSPASIKISVDELDQQRNIIEVPKLYSIDLDNQTLEQWKTQGNVSFSVTRPEHNIAISWPSVSYKAAQKEGSRHKRWAHWHTGLGGGGSGGGGSGGGGSFPTIPLSRLFDNAMLRAHRLHQLAFDTYQEFEEAYIPKEQKYSFLQNPQTSLCFSESIPTPSNREETQQKSNLELLRISLLLIQSWLEPVQFLRSVFANSLVYGASDSNVYDLLKDLEEGIQTLMGRLEDGSPRTGQIFKQTYSKFDTNSHNDDALLKNYGLLYCFRKDMDKVETFLRIVQCRSVEGSCGF

SEQ ID NO: 162 - protein, 451 aa, synthetic construct
  source 1..451: note = Description of Artificial Sequence: Synthetic polypeptide
MVEEALNIFDECRSPCSLTPEPGKPIQSKLSIPSDVVLDEGVLYYSMTINDEQNDIKDEDKGESIITIGEFATVRATRHYVNQDAPFGVIHLDITTENGTKTYSYNRKEGEFAINWLVPIGEDSPASIKISVDELDQQRNIIEVPKLYSIDLDNQTLEQWKTQGNVSFSVTRPEHNIAISWPSVSYKAAQKEGSRHKRWAHWHTGLALCWLVPMDAIYNYITQQNCTLGDNWFGGSYETVAGTPKGGGGSGGGGSGGGGSFPTIPLSRLFDNAMLRAHRLHQLAFDTYQEFEEAYIPKEQKYSFLQNPQTSLCFSESIPTPSNREETQQKSNLELLRISLLLIQSWLEPVQFLRSVFANSLVYGASDSNVYDLLKDLEEGIQTLMGRLEDGSPRTGQIFKQTYSKFDTNSHNDDALLKNYGLLYCFRKDMDKVETFLRIVQCRSVEGSCGF

SEQ ID NO: 163 - protein, 457 aa, synthetic construct
  source 1..457: note = Description of Artificial Sequence: Synthetic polypeptide
MVEEALNIFDECRSPCSLTPEPGKPIQSKLSIPSDVVLDEGVLYYSMTINDEQNDIKDEDKGESIITIGEFATVRATRHYVNQDAPFGVIHLDITTENGTKTYSYNRKEGEFAINWLVPIGEDSPASIKISVDELDQQRNIIEVPKLYSIDLDNQTLEQWKTQGNVSFSVTRPEHNIAISWPSVSYKAAQKEGSRHKRWAHWHTGLALCWLVPMDAIYNYITQQNCTLGDNWFGGSYETVAGTPKVITVKQGGGGSGGGGSGGGGSFPTIPLSRLFDNAMLRAHRLHQLAFDTYQEFEEAYIPKEQKYSFLQNPQTSLCFSESIPTPSNREETQQKSNLELLRISLLLIQSWLEPVQFLRSVFANSLVYGASDSNVYDLLKDLEEGIQTLMGRLEDGSPRTGQIFKQTYSKFDTNSHNDDALLKNYGLLYCFRKDMDKVETFLRIVQCRSVEGSCGF

SEQ ID NO: 164 - protein, 472 aa, synthetic construct
  source 1..472: note = Description of Artificial Sequence: Synthetic polypeptide
MVEEALNIFDECRSPCSLTPEPGKPIQSKLSIPSDVVLDEGVLYYSMTINDEQNDIKDEDKGESIITIGEFATVRATRHYVNQDAPFGVIHLDITTENGTKTYSYNRKEGEFAINWLVPIGEDSPASIKISVDELDQQRNIIEVPKLYSIDLDNQTLEQWKTQGNVSFSVTRPEHNIAISWPSVSYKAAQKEGSRHKRWAHWHTGLALCWLVPMDAIYNYITQQNCTLGDNWFGGSYETVAGTPKVITVKQGIEQKPVEQRIHFSKGGGGSGGGGSGGGGSFPTIPLSRLFDNAMLRAHRLHQLAFDTYQEFEEAYIPKEQKYSFLQNPQTSLCFSESIPTPSNREETQQKSNLELLRISLLLIQSWLEPVQFLRSVFANSLVYGASDSNVYDLLKDLEEGIQTLMGRLEDGSPRTGQIFKQTYSKFDTNSHNDDALLKNYGLLYCFRKDMDKVETFLRIVQCRSVEGSCGF

SEQ ID NO: 165 - protein, 354 aa, synthetic construct
  source 1..354: note = Description of Artificial Sequence: Synthetic polypeptide
GVLYYSMTINDEQNDIKDEDKGESIITIGEFATVRATRHYVNQDAPFGVIHLDITTENGTKTYSYNRKEGEFAINWLVPIGEDSPASIKISVDELDQQRNIIEVPKLYSIDLDNQTLEQWKTQGNVSFSVTRPEHNIAISWPSVSYKAGGGGSGGGGSGGGGSFPTIPLSRLFDNAMLRAHRLHQLAFDTYQEFEEAYIPKEQKYSFLQNPQTSLCFSESIPTPSNREETQQKSNLELLRISLLLIQSWLEPVQFLRSVFANSLVYGASDSNVYDLLKDLEEGIQTLMGRLEDGSPRTGQIFKQTYSKFDTNSHNDDALLKNYGLLYCFRKDMDKVETFLRIVQCRSVEGSCGF

SEQ ID NO: 166 - protein, 4 aa, unidentified
  source 1..4: note = Description of Unknown: Peptidase cleavage sequence
AAPF

SEQ ID NO: 167 - skipped

SEQ ID NO: 168 - protein, 4 aa, unidentified
  source 1..4: note = Description of Unknown: Peptidase cleavage sequence
AAPV

SEQ ID NO: 169-172 - skipped (4 entries)

SEQ ID NO: 173 - protein, 4 aa, unidentified
  source 1..4: note = Description of Unknown: Peptidase cleavage sequence
RQPR

SEQ ID NO: 174 - protein, 5 aa, unidentified
  source 1..5: note = Description of Unknown: Peptidase cleavage sequence
  VARIANT 5: note = MOD_RES - Any amino acid
YVADX

SEQ ID NO: 175-177 - skipped (3 entries)

SEQ ID NO: 178 - protein, 6 aa, unidentified
  source 1..6: note = Description of Unknown: Peptidase cleavage sequence
  VARIANT 6: note = MOD_RES - Any amino acid
ERTKRX

SEQ ID NO: 179 - protein, 5 aa, unidentified
  source 1..5: note = Description of Unknown: Peptidase cleavage sequence
  VARIANT 5: note = MOD_RES - Any amino acid
RVRRX

SEQ ID NO: 180 - protein, 5 aa, unidentified
  source 1..5: note = Description of Unknown: Peptidase cleavage sequence
  VARIANT 5: note = MOD_RES - Any amino acid
RVRRX

SEQ ID NO: 181 - protein, 6 aa, unidentified
  source 1..6: note = Description of Unknown: Peptidase cleavage sequence
  VARIANT 2: note = MOD_RES - Any amino acid
  VARIANT 6: note = MOD_RES - Any amino acid
PXWVPX

SEQ ID NO: 182-185 - skipped (4 entries)

SEQ ID NO: 186 - protein, 12 aa, unidentified
  source 1..12: note = Description of Unknown: Peptidase cleavage sequence
  VARIANT 10: note = MOD_RES - valine, alanine, or proline
  VARIANT 12: note = MOD_RES - serine, proline, or alanine
  REGION 1..12: note = SITE - Variant residues given in the sequence have no preference with respect to those in the annotations for variant positions
DRYIPFHLLXYX

SEQ ID NO: 187 - protein, 15 aa, synthetic construct
  source 1..15: note = Description of Artificial Sequence: Synthetic peptide
SGGGGSGKAGSRGLT

SEQ ID NO: 188 - protein, 15 aa, synthetic construct
  source 1..15: note = Description of Artificial Sequence: Synthetic peptide
SGGGGSGGGGLRQPR

SEQ ID NO: 189 - protein, 15 aa, synthetic construct
  source 1..15: note = Description of Artificial Sequence: Synthetic peptide
SGGGGSGKKVERFRY

SEQ ID NO: 190 - protein, 15 aa, synthetic construct
  source 1..15: note = Description of Artificial Sequence: Synthetic peptide
SGGGGSGGGGLMTPR

SEQ ID NO: 191 - protein, 15 aa, synthetic construct
  source 1..15: note = Description of Artificial Sequence: Synthetic peptide
SGGGGSGKAGSFSEG

SEQ ID NO: 192 - protein, 15 aa, synthetic construct
  source 1..15: note = Description of Artificial Sequence: Synthetic peptide
SGGGGSGKAGSAAPF

SEQ ID NO: 193 - protein, 15 aa, synthetic construct
  source 1..15: note = Description of Artificial Sequence: Synthetic peptide
GGGGSGGGENLYFQS

SEQ ID NO: 194 - protein, 12 aa, synthetic construct
  source 1..12: note = Description of Artificial Sequence: Synthetic peptide
VSWKTWFPNLAV

SEQ ID NO: 195 - protein, 12 aa, synthetic construct
  source 1..12: note = Description of Artificial Sequence: Synthetic peptide
YSPFHKWFPSMH

SEQ ID NO: 196 - protein, 12 aa, synthetic construct
  source 1..12: note = Description of Artificial Sequence: Synthetic peptide
IPQVWRDWFKLP

SEQ ID NO: 197 - protein, 12 aa, synthetic construct
  source 1..12: note = Description of Artificial Sequence: Synthetic peptide
FPAWFTKLYPRT

SEQ ID NO: 198 - protein, 12 aa, synthetic construct
  source 1..12: note = Description of Artificial Sequence: Synthetic peptide
QINTAKWWKTHF

SEQ ID NO: 199 - protein, 12 aa, synthetic construct
  source 1..12: note = Description of Artificial Sequence: Synthetic peptide
DASKALRSSGMP

SEQ ID NO: 200 - protein, 6 aa, synthetic construct
  source 1..6: note = Description of Artificial Sequence: Synthetic peptide
WKTWFP

SEQ ID NO: 201 - protein, 15 aa, synthetic construct
  source 1..15: note = Description of Artificial Sequence: Synthetic peptide
SGGGGWKTWFPRGLT

SEQ ID NO: 202 - protein, 15 aa, synthetic construct
  source 1..15: note = Description of Artificial Sequence: Synthetic peptide
SGGGGWKTWFPRQPR

SEQ ID NO: 203 - protein, 15 aa, synthetic construct
  source 1..15: note = Description of Artificial Sequence: Synthetic peptide
SGGGGWKTWFPRFRY

SEQ ID NO: 204 - protein, 15 aa, synthetic construct
  source 1..15: note = Description of Artificial Sequence: Synthetic peptide
SGGGGWKTWFPMTPR

SEQ ID NO: 205 - protein, 15 aa, synthetic construct
  source 1..15: note = Description of Artificial Sequence: Synthetic peptide
SGGGGWKTWFPFSEG

SEQ ID NO: 206 - protein, 15 aa, synthetic construct
  source 1..15: note = Description of Artificial Sequence: Synthetic peptide
SGGGGWKTWFPAAPF

SEQ ID NO: 207 - protein, 5 aa, synthetic construct
  source 1..5: note = Description of Artificial Sequence: Synthetic peptide
GTGGS

SEQ ID NO: 208 - protein, 5 aa, synthetic construct
  source 1..5: note = Description of Artificial Sequence: Synthetic peptide
GGGGS

SEQ ID NO: 209 - protein, 10 aa, synthetic construct
  source 1..10: note = Description of Artificial Sequence: Synthetic peptide
GGGGSGGGGS

SEQ ID NO: 210 - protein, 15 aa, synthetic construct
  source 1..15: note = Description of Artificial Sequence: Synthetic peptide
GGGGSGGGGSGGGGS

SEQ ID NO: 211 - protein, 8 aa, synthetic construct
  source 1..8: note = Description of Artificial Sequence: Synthetic peptide
GGGGSGGG

SEQ ID NO: 212 - protein, 50 aa, synthetic construct
  source 1..50: note = Description of Artificial Sequence: Synthetic polypeptide
  VARIANT 1..50: note = SITE - This sequence may encompass 1-10 GGGGS repeating units
GGGGSGGGGSGGGGSGGGGSGGGGSGGGGSGGGGSGGGGSGGGGSGGGGS

SEQ ID NO: 213 - protein, 20 aa, synthetic construct
  source 1..20: note = Description of Artificial Sequence: Synthetic peptide
  VARIANT 1..20: note = SITE - This sequence may encompass 1-10 GS repeating units
GSGSGSGSGSGSGSGSGSGS

SEQ ID NO: 214 - protein, 191 aa, Homo sapiens [sequence omitted]

SEQ ID NO: 215 - protein, 87 aa, unidentified
  source 1..87: note = Description of Unknown: GPL-1 agonist peptide
MKIILWLCVFGLFLATLFPISWQMPVESGLSSEDSASSESFASKIKRHGEGTFTSDLSKQMEEEAVRLFIEWLKNGGPSSGAPPPSG

SEQ ID NO: 216 - protein, 110 aa, unidentified
  source 1..110: note = Description of Unknown: Insulin peptide
MALWMRLLPLLALLALWGPDPAAAFVNQHLCGSHLVEALYLVCGERGFFYTPKTRREAEDLQVGQVELGGGPGAGSLQPLALEGSLQKRGIVEQCCTSICSLYQLENYCN

SEQ ID NO: 217 - protein, 178 aa, Homo sapiens
MHSSALLCCLVLLTGVRASPGQGTQSENSCTHFPGNLPNMLRDLRDAFSRVKTFFQMKDQLDNLLLKESLLEDFKGYLGCQALSEMIQFYLEEVMPQAENQDPDIKAHVNSLGENLKTLRLRLRRCHRFLPCENKSKAVEQVKNAFNKLQEKGIYKAMSEFDIFINYIEAYMTMKIRN

SEQ ID NO: 218 - protein, 179 aa, Homo sapiens
MAALQKSVSSFLMGTLATSCLLLLALLVQGGAAAPISSHCRLDKSNFQQPYITNRTFMLAKEASLADNNTDVRLIGEKLFHGVSMSERCYLMKQVLNFTLEEVLFPQSDRFQPYMQEVVPFLARLSNRLSTCHIEGDDLHIQRNVQKLKDTVKKLGESGEIKAIGELDLLFMSLRNACI

SEQ ID NO: 219 - protein, 71 aa, unidentified
  source 1..71: note = Description of Unknown: ExtB polypeptide
MKKNIAFLLASMFVFSIATNAYASTQSNKKDLCEHYRQIAKESCKKGFLGVRDGTAGACFGAQIMVAAKGC

SEQ ID NO: 220 - protein, 225 aa, unidentified
  source 1..225: note = Description of Unknown: Red Fluorescent Protein (RFP) sequence
MRSSKNVIKEFMRFKVRMEGTVNGHEFEIEGEGEGRPYEGHNTVKLKVTKGGPLPFAWDILSPQFQYGSKVYVKHPADIPDYKKLSFPEGFKWERVMNFEDGGVVTVTQDSSLQDGCFIYKVKFIGVNFPSDGPVMQKKTMGWEASTERLYPRDGVLKGEIHKALKLKDGGHYLVEFKSIYMAKKPVQLPGYYYVDSKLDITSHNEDYTIVEQYERTEGRHHLFL

SEQ ID NO: 221 - protein, 281 aa, synthetic construct
  source 1..281: note = Description of Artificial Sequence: Synthetic polypeptide
MVEEALNIFDECRSPCSLTPEPGKPIQSKLSIPSDVVLDEGVLYYSMTINDEQNDIKDEDKGESIITIGEFATVRATRHYVNQDAPFGVIHLDITTENGTKTYSYNRKEGEFAINWLVPIGEDSPASIKISVDELDQQRNIIEVPKLYSIDLDNQTLEQWKTQGNVSFSVTRPEHNIAISWPSVSYKAAQKEGSRHKRWAHWHTGLALCWLVPMDAIYNYITQQNCTLGDNWFGGSYETVAGTPKVITVKQGIEQKPVEQRIHFSKGGGGSGGGGSGGGGS